European Patent Application EP 4 663 199 A1, published December 17, 2025. Title: FUSION POLYPEPTIDE AND LIPONANOPARTICLE COMPRISING THE SAME. Applicant: Strike Pharma AB. Application EP, filed June 12, 2024. The sequence listing filed with the application follows.

SEQUENCE LISTING (453 sequences)

SEQ ID NO: 1 - protein, 9 aa, synthetic construct
  SITE 8: note = X = K, L or H
  SITE 9: note = X = K or absent
FIGITELXX

SEQ ID NO: 2 - protein, 9 aa, synthetic construct
FIGITELKK

SEQ ID NO: 3 - protein, 9 aa, synthetic construct
FIGITELLK

SEQ ID NO: 4 - protein, 9 aa, synthetic construct
FIGITELHK

SEQ ID NO: 5 - protein, 8 aa, synthetic construct
FIGITELK

SEQ ID NO: 6 - protein, 8 aa, synthetic construct
FIGITELL

SEQ ID NO: 7 - protein, 8 aa, synthetic construct
FIGITELH

SEQ ID NO: 8 - skipped

SEQ ID NO: 9 - protein, 5 aa, synthetic construct
GGGGS

SEQ ID NO: 10 - protein, 10 aa, synthetic construct
GGGGSGGGGS

SEQ ID NO: 11 - protein, 15 aa, synthetic construct
GGGGSGGGGSGGGGS

SEQ ID NO: 12 - protein, 5 aa, synthetic construct
EAAAK

SEQ ID NO: 13 - protein, 10 aa, synthetic construct
EAAAKEAAAK

SEQ ID NO: 14 - protein, 15 aa, synthetic construct
EAAAKEAAAKEAAAK

SEQ ID NO: 15-17 - skipped (3 entries)

SEQ ID NO: 18 - protein, 299 aa, synthetic construct
KVEQAVETEPEPELRQQTEWQSGQRWELALGRFWDYLRWVQTLSEQVQEELLSSQVTQELRALMDETMKELKAYKSELEEQLTPVAEETRARLSKELQAAQARLGADMEDVCGRLVQYRGEVQAMLGQSTEELRVSLASHLRKLRKRLLRDADDLQKCLAVYQAGAREGAERGLSAIRERLGPLVEQGRVRAATVGSLAGQPLQERAQAWGERLRARMEEMGSRTRDRLDEVKEQVAEVRAKLEEQAQQIRLQAEAFQARLKSWFEPLVEDMQRQWAGLVEKVQAAVGTSAAPVPSDNH

SEQ ID NO: 19 - protein, 109 aa, synthetic construct
RAATVGSLAGQPLQERAQAWGERLRARMEEMGSRTRDRLDEVKEQVAEVRAKLEEQAQQIRLQAEAFQARLKSWFEPLVEDMQRQWAGLVEKVQAAVGTSAAPVPSDNH

SEQ ID NO: 20 - protein, 136 aa, synthetic construct
AGAREGAERGLSAIRERLGPLVEQGRVRAATVGSLAGQPLQERAQAWGERLRARMEEMGSRTRDRLDEVKEQVAEVRAKLEEQAQQIRLQAEAFQARLKSWFEPLVEDMQRQWAGLVEKVQAAVGTSAAPVPSDNH

SEQ ID NO: 21 - protein, 256 aa, synthetic construct
SEQVQEELLSSQVTQELRALMDETMKELKAYKSELEEQLTPVAEETRARLSKELQAAQARLGADMEDVCGRLVQYRGEVQAMLGQSTEELRVSLASHLRKLRKRLLRDADDLQKCLAVYQAGAREGAERGLSAIRERLGPLVEQGRVRAATVGSLAGQPLQERAQAWGERLRARMEEMGSRTRDRLDEVKEQVAEVRAKLEEQAQQIRLQAEAFQARLKSWFEPLVEDMQRQWAGLVEKVQAAVGTSAAPVPSDNH

SEQ ID NO: 22 - protein, 246 aa, synthetic construct
SQVTQELRALMDETMKELKAYKSELEEQLTPVAEETRARLSKELQAAQARLGADMEDVCGRLVQYRGEVQAMLGQSTEELRVSLASHLRKLRKRLLRDADDLQKCLAVYQAGAREGAERGLSAIRERLGPLVEQGRVRAATVGSLAGQPLQERAQAWGERLRARMEEMGSRTRDRLDEVKEQVAEVRAKLEEQAQQIRLQAEAFQARLKSWFEPLVEDMQRQWAGLVEKVQAAVGTSAAPVPSDNH

SEQ ID NO: 23-32 - skipped (10 entries)

SEQ ID NO: 33 - protein, 308 aa, synthetic construct
FIGITELKKKVEQAVETEPEPELRQQTEWQSGQRWELALGRFWDYLRWVQTLSEQVQEELLSSQVTQELRALMDETMKELKAYKSELEEQLTPVAEETRARLSKELQAAQARLGADMEDVCGRLVQYRGEVQAMLGQSTEELRVSLASHLRKLRKRLLRDADDLQKCLAVYQAGAREGAERGLSAIRERLGPLVEQGRVRAATVGSLAGQPLQERAQAWGERLRARMEEMGSRTRDRLDEVKEQVAEVRAKLEEQAQQIRLQAEAFQARLKSWFEPLVEDMQRQWAGLVEKVQAAVGTSAAPVPSDNH

SEQ ID NO: 34 - protein, 313 aa, synthetic construct
FIGITELKKGGGGSKVEQAVETEPEPELRQQTEWQSGQRWELALGRFWDYLRWVQTLSEQVQEELLSSQVTQELRALMDETMKELKAYKSELEEQLTPVAEETRARLSKELQAAQARLGADMEDVCGRLVQYRGEVQAMLGQSTEELRVSLASHLRKLRKRLLRDADDLQKCLAVYQAGAREGAERGLSAIRERLGPLVEQGRVRAATVGSLAGQPLQERAQAWGERLRARMEEMGSRTRDRLDEVKEQVAEVRAKLEEQAQQIRLQAEAFQARLKSWFEPLVEDMQRQWAGLVEKVQAAVGTSAAPVPSDNH

SEQ ID NO: 35 - protein, 318 aa, synthetic construct
FIGITELKKGGGGSGGGGSKVEQAVETEPEPELRQQTEWQSGQRWELALGRFWDYLRWVQTLSEQVQEELLSSQVTQELRALMDETMKELKAYKSELEEQLTPVAEETRARLSKELQAAQARLGADMEDVCGRLVQYRGEVQAMLGQSTEELRVSLASHLRKLRKRLLRDADDLQKCLAVYQAGAREGAERGLSAIRERLGPLVEQGRVRAATVGSLAGQPLQERAQAWGERLRARMEEMGSRTRDRLDEVKEQVAEVRAKLEEQAQQIRLQAEAFQARLKSWFEPLVEDMQRQWAGLVEKVQAAVGTSAAPVPSDNH

SEQ ID NO: 36 - protein, 323 aa, synthetic construct
FIGITELKKGGGGSGGGGSGGGGSKVEQAVETEPEPELRQQTEWQSGQRWELALGRFWDYLRWVQTLSEQVQEELLSSQVTQELRALMDETMKELKAYKSELEEQLTPVAEETRARLSKELQAAQARLGADMEDVCGRLVQYRGEVQAMLGQSTEELRVSLASHLRKLRKRLLRDADDLQKCLAVYQAGAREGAERGLSAIRERLGPLVEQGRVRAATVGSLAGQPLQERAQAWGERLRARMEEMGSRTRDRLDEVKEQVAEVRAKLEEQAQQIRLQAEAFQARLKSWFEPLVEDMQRQWAGLVEKVQAAVGTSAAPVPSDNH

SEQ ID NO: 37 - protein, 313 aa, synthetic construct
FIGITELKKEAAAKKVEQAVETEPEPELRQQTEWQSGQRWELALGRFWDYLRWVQTLSEQVQEELLSSQVTQELRALMDETMKELKAYKSELEEQLTPVAEETRARLSKELQAAQARLGADMEDVCGRLVQYRGEVQAMLGQSTEELRVSLASHLRKLRKRLLRDADDLQKCLAVYQAGAREGAERGLSAIRERLGPLVEQGRVRAATVGSLAGQPLQERAQAWGERLRARMEEMGSRTRDRLDEVKEQVAEVRAKLEEQAQQIRLQAEAFQARLKSWFEPLVEDMQRQWAGLVEKVQAAVGTSAAPVPSDNH

SEQ ID NO: 38 - protein, 318 aa, synthetic construct
FIGITELKKEAAAKEAAAKKVEQAVETEPEPELRQQTEWQSGQRWELALGRFWDYLRWVQTLSEQVQEELLSSQVTQELRALMDETMKELKAYKSELEEQLTPVAEETRARLSKELQAAQARLGADMEDVCGRLVQYRGEVQAMLGQSTEELRVSLASHLRKLRKRLLRDADDLQKCLAVYQAGAREGAERGLSAIRERLGPLVEQGRVRAATVGSLAGQPLQERAQAWGERLRARMEEMGSRTRDRLDEVKEQVAEVRAKLEEQAQQIRLQAEAFQARLKSWFEPLVEDMQRQWAGLVEKVQAAVGTSAAPVPSDNH

SEQ ID NO: 39 - protein, 323 aa, synthetic construct
FIGITELKKEAAAKEAAAKEAAAKKVEQAVETEPEPELRQQTEWQSGQRWELALGRFWDYLRWVQTLSEQVQEELLSSQVTQELRALMDETMKELKAYKSELEEQLTPVAEETRARLSKELQAAQARLGADMEDVCGRLVQYRGEVQAMLGQSTEELRVSLASHLRKLRKRLLRDADDLQKCLAVYQAGAREGAERGLSAIRERLGPLVEQGRVRAATVGSLAGQPLQERAQAWGERLRARMEEMGSRTRDRLDEVKEQVAEVRAKLEEQAQQIRLQAEAFQARLKSWFEPLVEDMQRQWAGLVEKVQAAVGTSAAPVPSDNH

SEQ ID NO: 40 - protein, 311 aa, synthetic construct
FIGITELKKGGSKVEQAVETEPEPELRQQTEWQSGQRWELALGRFWDYLRWVQTLSEQVQEELLSSQVTQELRALMDETMKELKAYKSELEEQLTPVAEETRARLSKELQAAQARLGADMEDVCGRLVQYRGEVQAMLGQSTEELRVSLASHLRKLRKRLLRDADDLQKCLAVYQAGAREGAERGLSAIRERLGPLVEQGRVRAATVGSLAGQPLQERAQAWGERLRARMEEMGSRTRDRLDEVKEQVAEVRAKLEEQAQQIRLQAEAFQARLKSWFEPLVEDMQRQWAGLVEKVQAAVGTSAAPVPSDNH

SEQ ID NO: 41 - protein, 311 aa, synthetic construct
FIGITELKKAAAKVEQAVETEPEPELRQQTEWQSGQRWELALGRFWDYLRWVQTLSEQVQEELLSSQVTQELRALMDETMKELKAYKSELEEQLTPVAEETRARLSKELQAAQARLGADMEDVCGRLVQYRGEVQAMLGQSTEELRVSLASHLRKLRKRLLRDADDLQKCLAVYQAGAREGAERGLSAIRERLGPLVEQGRVRAATVGSLAGQPLQERAQAWGERLRARMEEMGSRTRDRLDEVKEQVAEVRAKLEEQAQQIRLQAEAFQARLKSWFEPLVEDMQRQWAGLVEKVQAAVGTSAAPVPSDNH

SEQ ID NO: 42 - protein, 311 aa, synthetic construct
FIGITELKKAAYKVEQAVETEPEPELRQQTEWQSGQRWELALGRFWDYLRWVQTLSEQVQEELLSSQVTQELRALMDETMKELKAYKSELEEQLTPVAEETRARLSKELQAAQARLGADMEDVCGRLVQYRGEVQAMLGQSTEELRVSLASHLRKLRKRLLRDADDLQKCLAVYQAGAREGAERGLSAIRERLGPLVEQGRVRAATVGSLAGQPLQERAQAWGERLRARMEEMGSRTRDRLDEVKEQVAEVRAKLEEQAQQIRLQAEAFQARLKSWFEPLVEDMQRQWAGLVEKVQAAVGTSAAPVPSDNH

SEQ ID NO: 43 - protein, 308 aa, synthetic construct
FIGITELLKKVEQAVETEPEPELRQQTEWQSGQRWELALGRFWDYLRWVQTLSEQVQEELLSSQVTQELRALMDETMKELKAYKSELEEQLTPVAEETRARLSKELQAAQARLGADMEDVCGRLVQYRGEVQAMLGQSTEELRVSLASHLRKLRKRLLRDADDLQKCLAVYQAGAREGAERGLSAIRERLGPLVEQGRVRAATVGSLAGQPLQERAQAWGERLRARMEEMGSRTRDRLDEVKEQVAEVRAKLEEQAQQIRLQAEAFQARLKSWFEPLVEDMQRQWAGLVEKVQAAVGTSAAPVPSDNH

SEQ ID NO: 44 - protein, 313 aa, synthetic construct
FIGITELLKGGGGSKVEQAVETEPEPELRQQTEWQSGQRWELALGRFWDYLRWVQTLSEQVQEELLSSQVTQELRALMDETMKELKAYKSELEEQLTPVAEETRARLSKELQAAQARLGADMEDVCGRLVQYRGEVQAMLGQSTEELRVSLASHLRKLRKRLLRDADDLQKCLAVYQAGAREGAERGLSAIRERLGPLVEQGRVRAATVGSLAGQPLQERAQAWGERLRARMEEMGSRTRDRLDEVKEQVAEVRAKLEEQAQQIRLQAEAFQARLKSWFEPLVEDMQRQWAGLVEKVQAAVGTSAAPVPSDNH

SEQ ID NO: 45 - protein, 318 aa, synthetic construct
FIGITELLKGGGGSGGGGSKVEQAVETEPEPELRQQTEWQSGQRWELALGRFWDYLRWVQTLSEQVQEELLSSQVTQELRALMDETMKELKAYKSELEEQLTPVAEETRARLSKELQAAQARLGADMEDVCGRLVQYRGEVQAMLGQSTEELRVSLASHLRKLRKRLLRDADDLQKCLAVYQAGAREGAERGLSAIRERLGPLVEQGRVRAATVGSLAGQPLQERAQAWGERLRARMEEMGSRTRDRLDEVKEQVAEVRAKLEEQAQQIRLQAEAFQARLKSWFEPLVEDMQRQWAGLVEKVQAAVGTSAAPVPSDNH

SEQ ID NO: 46 - protein, 323 aa, synthetic construct
FIGITELLKGGGGSGGGGSGGGGSKVEQAVETEPEPELRQQTEWQSGQRWELALGRFWDYLRWVQTLSEQVQEELLSSQVTQELRALMDETMKELKAYKSELEEQLTPVAEETRARLSKELQAAQARLGADMEDVCGRLVQYRGEVQAMLGQSTEELRVSLASHLRKLRKRLLRDADDLQKCLAVYQAGAREGAERGLSAIRERLGPLVEQGRVRAATVGSLAGQPLQERAQAWGERLRARMEEMGSRTRDRLDEVKEQVAEVRAKLEEQAQQIRLQAEAFQARLKSWFEPLVEDMQRQWAGLVEKVQAAVGTSAAPVPSDNH

SEQ ID NO: 47 - protein, 313 aa, synthetic construct
FIGITELLKEAAAKKVEQAVETEPEPELRQQTEWQSGQRWELALGRFWDYLRWVQTLSEQVQEELLSSQVTQELRALMDETMKELKAYKSELEEQLTPVAEETRARLSKELQAAQARLGADMEDVCGRLVQYRGEVQAMLGQSTEELRVSLASHLRKLRKRLLRDADDLQKCLAVYQAGAREGAERGLSAIRERLGPLVEQGRVRAATVGSLAGQPLQERAQAWGERLRARMEEMGSRTRDRLDEVKEQVAEVRAKLEEQAQQIRLQAEAFQARLKSWFEPLVEDMQRQWAGLVEKVQAAVGTSAAPVPSDNH

SEQ ID NO: 48 - protein, 318 aa, synthetic construct
FIGITELLKEAAAKEAAAKKVEQAVETEPEPELRQQTEWQSGQRWELALGRFWDYLRWVQTLSEQVQEELLSSQVTQELRALMDETMKELKAYKSELEEQLTPVAEETRARLSKELQAAQARLGADMEDVCGRLVQYRGEVQAMLGQSTEELRVSLASHLRKLRKRLLRDADDLQKCLAVYQAGAREGAERGLSAIRERLGPLVEQGRVRAATVGSLAGQPLQERAQAWGERLRARMEEMGSRTRDRLDEVKEQVAEVRAKLEEQAQQIRLQAEAFQARLKSWFEPLVEDMQRQWAGLVEKVQAAVGTSAAPVPSDNH

SEQ ID NO: 49 - protein, 323 aa, synthetic construct
FIGITELLKEAAAKEAAAKEAAAKKVEQAVETEPEPELRQQTEWQSGQRWELALGRFWDYLRWVQTLSEQVQEELLSSQVTQELRALMDETMKELKAYKSELEEQLTPVAEETRARLSKELQAAQARLGADMEDVCGRLVQYRGEVQAMLGQSTEELRVSLASHLRKLRKRLLRDADDLQKCLAVYQAGAREGAERGLSAIRERLGPLVEQGRVRAATVGSLAGQPLQERAQAWGERLRARMEEMGSRTRDRLDEVKEQVAEVRAKLEEQAQQIRLQAEAFQARLKSWFEPLVEDMQRQWAGLVEKVQAAVGTSAAPVPSDNH

SEQ ID NO: 50 - protein, 311 aa, synthetic construct
FIGITELLKGGSKVEQAVETEPEPELRQQTEWQSGQRWELALGRFWDYLRWVQTLSEQVQEELLSSQVTQELRALMDETMKELKAYKSELEEQLTPVAEETRARLSKELQAAQARLGADMEDVCGRLVQYRGEVQAMLGQSTEELRVSLASHLRKLRKRLLRDADDLQKCLAVYQAGAREGAERGLSAIRERLGPLVEQGRVRAATVGSLAGQPLQERAQAWGERLRARMEEMGSRTRDRLDEVKEQVAEVRAKLEEQAQQIRLQAEAFQARLKSWFEPLVEDMQRQWAGLVEKVQAAVGTSAAPVPSDNH

SEQ ID NO: 51 - protein, 311 aa, synthetic construct
FIGITELLKAAAKVEQAVETEPEPELRQQTEWQSGQRWELALGRFWDYLRWVQTLSEQVQEELLSSQVTQELRALMDETMKELKAYKSELEEQLTPVAEETRARLSKELQAAQARLGADMEDVCGRLVQYRGEVQAMLGQSTEELRVSLASHLRKLRKRLLRDADDLQKCLAVYQAGAREGAERGLSAIRERLGPLVEQGRVRAATVGSLAGQPLQERAQAWGERLRARMEEMGSRTRDRLDEVKEQVAEVRAKLEEQAQQIRLQAEAFQARLKSWFEPLVEDMQRQWAGLVEKVQAAVGTSAAPVPSDNH

SEQ ID NO: 52 - protein, 311 aa, synthetic construct
FIGITELLKAAYKVEQAVETEPEPELRQQTEWQSGQRWELALGRFWDYLRWVQTLSEQVQEELLSSQVTQELRALMDETMKELKAYKSELEEQLTPVAEETRARLSKELQAAQARLGADMEDVCGRLVQYRGEVQAMLGQSTEELRVSLASHLRKLRKRLLRDADDLQKCLAVYQAGAREGAERGLSAIRERLGPLVEQGRVRAATVGSLAGQPLQERAQAWGERLRARMEEMGSRTRDRLDEVKEQVAEVRAKLEEQAQQIRLQAEAFQARLKSWFEPLVEDMQRQWAGLVEKVQAAVGTSAAPVPSDNH

SEQ ID NO: 53 - protein, 308 aa, synthetic construct
FIGITELHKKVEQAVETEPEPELRQQTEWQSGQRWELALGRFWDYLRWVQTLSEQVQEELLSSQVTQELRALMDETMKELKAYKSELEEQLTPVAEETRARLSKELQAAQARLGADMEDVCGRLVQYRGEVQAMLGQSTEELRVSLASHLRKLRKRLLRDADDLQKCLAVYQAGAREGAERGLSAIRERLGPLVEQGRVRAATVGSLAGQPLQERAQAWGERLRARMEEMGSRTRDRLDEVKEQVAEVRAKLEEQAQQIRLQAEAFQARLKSWFEPLVEDMQRQWAGLVEKVQAAVGTSAAPVPSDNH

SEQ ID NO: 54 - protein, 313 aa, synthetic construct
FIGITELHKGGGGSKVEQAVETEPEPELRQQTEWQSGQRWELALGRFWDYLRWVQTLSEQVQEELLSSQVTQELRALMDETMKELKAYKSELEEQLTPVAEETRARLSKELQAAQARLGADMEDVCGRLVQYRGEVQAMLGQSTEELRVSLASHLRKLRKRLLRDADDLQKCLAVYQAGAREGAERGLSAIRERLGPLVEQGRVRAATVGSLAGQPLQERAQAWGERLRARMEEMGSRTRDRLDEVKEQVAEVRAKLEEQAQQIRLQAEAFQARLKSWFEPLVEDMQRQWAGLVEKVQAAVGTSAAPVPSDNH

SEQ ID NO: 55 - protein, 318 aa, synthetic construct
FIGITELHKGGGGSGGGGSKVEQAVETEPEPELRQQTEWQSGQRWELALGRFWDYLRWVQTLSEQVQEELLSSQVTQELRALMDETMKELKAYKSELEEQLTPVAEETRARLSKELQAAQARLGADMEDVCGRLVQYRGEVQAMLGQSTEELRVSLASHLRKLRKRLLRDADDLQKCLAVYQAGAREGAERGLSAIRERLGPLVEQGRVRAATVGSLAGQPLQERAQAWGERLRARMEEMGSRTRDRLDEVKEQVAEVRAKLEEQAQQIRLQAEAFQARLKSWFEPLVEDMQRQWAGLVEKVQAAVGTSAAPVPSDNH

SEQ ID NO: 56 - protein, 323 aa, synthetic construct
FIGITELHKGGGGSGGGGSGGGGSKVEQAVETEPEPELRQQTEWQSGQRWELALGRFWDYLRWVQTLSEQVQEELLSSQVTQELRALMDETMKELKAYKSELEEQLTPVAEETRARLSKELQAAQARLGADMEDVCGRLVQYRGEVQAMLGQSTEELRVSLASHLRKLRKRLLRDADDLQKCLAVYQAGAREGAERGLSAIRERLGPLVEQGRVRAATVGSLAGQPLQERAQAWGERLRARMEEMGSRTRDRLDEVKEQVAEVRAKLEEQAQQIRLQAEAFQARLKSWFEPLVEDMQRQWAGLVEKVQAAVGTSAAPVPSDNH

SEQ ID NO: 57 - protein, 313 aa, synthetic construct
FIGITELHKEAAAKKVEQAVETEPEPELRQQTEWQSGQRWELALGRFWDYLRWVQTLSEQVQEELLSSQVTQELRALMDETMKELKAYKSELEEQLTPVAEETRARLSKELQAAQARLGADMEDVCGRLVQYRGEVQAMLGQSTEELRVSLASHLRKLRKRLLRDADDLQKCLAVYQAGAREGAERGLSAIRERLGPLVEQGRVRAATVGSLAGQPLQERAQAWGERLRARMEEMGSRTRDRLDEVKEQVAEVRAKLEEQAQQIRLQAEAFQARLKSWFEPLVEDMQRQWAGLVEKVQAAVGTSAAPVPSDNH

SEQ ID NO: 58 - protein, 318 aa, synthetic construct
FIGITELHKEAAAKEAAAKKVEQAVETEPEPELRQQTEWQSGQRWELALGRFWDYLRWVQTLSEQVQEELLSSQVTQELRALMDETMKELKAYKSELEEQLTPVAEETRARLSKELQAAQARLGADMEDVCGRLVQYRGEVQAMLGQSTEELRVSLASHLRKLRKRLLRDADDLQKCLAVYQAGAREGAERGLSAIRERLGPLVEQGRVRAATVGSLAGQPLQERAQAWGERLRARMEEMGSRTRDRLDEVKEQVAEVRAKLEEQAQQIRLQAEAFQARLKSWFEPLVEDMQRQWAGLVEKVQAAVGTSAAPVPSDNH

SEQ ID NO: 59 - protein, 323 aa, synthetic construct
FIGITELHKEAAAKEAAAKEAAAKKVEQAVETEPEPELRQQTEWQSGQRWELALGRFWDYLRWVQTLSEQVQEELLSSQVTQELRALMDETMKELKAYKSELEEQLTPVAEETRARLSKELQAAQARLGADMEDVCGRLVQYRGEVQAMLGQSTEELRVSLASHLRKLRKRLLRDADDLQKCLAVYQAGAREGAERGLSAIRERLGPLVEQGRVRAATVGSLAGQPLQERAQAWGERLRARMEEMGSRTRDRLDEVKEQVAEVRAKLEEQAQQIRLQAEAFQARLKSWFEPLVEDMQRQWAGLVEKVQAAVGTSAAPVPSDNH

SEQ ID NO: 60 - protein, 311 aa, synthetic construct
FIGITELHKGGSKVEQAVETEPEPELRQQTEWQSGQRWELALGRFWDYLRWVQTLSEQVQEELLSSQVTQELRALMDETMKELKAYKSELEEQLTPVAEETRARLSKELQAAQARLGADMEDVCGRLVQYRGEVQAMLGQSTEELRVSLASHLRKLRKRLLRDADDLQKCLAVYQAGAREGAERGLSAIRERLGPLVEQGRVRAATVGSLAGQPLQERAQAWGERLRARMEEMGSRTRDRLDEVKEQVAEVRAKLEEQAQQIRLQAEAFQARLKSWFEPLVEDMQRQWAGLVEKVQAAVGTSAAPVPSDNH

SEQ ID NO: 61 - protein, 311 aa, synthetic construct
FIGITELHKAAAKVEQAVETEPEPELRQQTEWQSGQRWELALGRFWDYLRWVQTLSEQVQEELLSSQVTQELRALMDETMKELKAYKSELEEQLTPVAEETRARLSKELQAAQARLGADMEDVCGRLVQYRGEVQAMLGQSTEELRVSLASHLRKLRKRLLRDADDLQKCLAVYQAGAREGAERGLSAIRERLGPLVEQGRVRAATVGSLAGQPLQERAQAWGERLRARMEEMGSRTRDRLDEVKEQVAEVRAKLEEQAQQIRLQAEAFQARLKSWFEPLVEDMQRQWAGLVEKVQAAVGTSAAPVPSDNH

SEQ ID NO: 62 - protein, 311 aa, synthetic construct
FIGITELHKAAYKVEQAVETEPEPELRQQTEWQSGQRWELALGRFWDYLRWVQTLSEQVQEELLSSQVTQELRALMDETMKELKAYKSELEEQLTPVAEETRARLSKELQAAQARLGADMEDVCGRLVQYRGEVQAMLGQSTEELRVSLASHLRKLRKRLLRDADDLQKCLAVYQAGAREGAERGLSAIRERLGPLVEQGRVRAATVGSLAGQPLQERAQAWGERLRARMEEMGSRTRDRLDEVKEQVAEVRAKLEEQAQQIRLQAEAFQARLKSWFEPLVEDMQRQWAGLVEKVQAAVGTSAAPVPSDNH

SEQ ID NO: 63-73 - skipped (11 entries)

SEQ ID NO: 74 - protein, 118 aa, synthetic construct
FIGITELKKRAATVGSLAGQPLQERAQAWGERLRARMEEMGSRTRDRLDEVKEQVAEVRAKLEEQAQQIRLQAEAFQARLKSWFEPLVEDMQRQWAGLVEKVQAAVGTSAAPVPSDNH

SEQ ID NO: 75 - protein, 123 aa, synthetic construct
FIGITELKKGGGGSRAATVGSLAGQPLQERAQAWGERLRARMEEMGSRTRDRLDEVKEQVAEVRAKLEEQAQQIRLQAEAFQARLKSWFEPLVEDMQRQWAGLVEKVQAAVGTSAAPVPSDNH

SEQ ID NO: 76 - protein, 128 aa, synthetic construct
FIGITELKKGGGGSGGGGSRAATVGSLAGQPLQERAQAWGERLRARMEEMGSRTRDRLDEVKEQVAEVRAKLEEQAQQIRLQAEAFQARLKSWFEPLVEDMQRQWAGLVEKVQAAVGTSAAPVPSDNH

SEQ ID NO: 77 - protein, 133 aa, synthetic construct
FIGITELKKGGGGSGGGGSGGGGSRAATVGSLAGQPLQERAQAWGERLRARMEEMGSRTRDRLDEVKEQVAEVRAKLEEQAQQIRLQAEAFQARLKSWFEPLVEDMQRQWAGLVEKVQAAVGTSAAPVPSDNH

SEQ ID NO: 78 - protein, 123 aa, synthetic construct
FIGITELKKEAAAKRAATVGSLAGQPLQERAQAWGERLRARMEEMGSRTRDRLDEVKEQVAEVRAKLEEQAQQIRLQAEAFQARLKSWFEPLVEDMQRQWAGLVEKVQAAVGTSAAPVPSDNH

SEQ ID NO: 79 - protein, 128 aa, synthetic construct
FIGITELKKEAAAKEAAAKRAATVGSLAGQPLQERAQAWGERLRARMEEMGSRTRDRLDEVKEQVAEVRAKLEEQAQQIRLQAEAFQARLKSWFEPLVEDMQRQWAGLVEKVQAAVGTSAAPVPSDNH

SEQ ID NO: 80 - protein, 133 aa, synthetic construct
FIGITELKKEAAAKEAAAKEAAAKRAATVGSLAGQPLQERAQAWGERLRARMEEMGSRTRDRLDEVKEQVAEVRAKLEEQAQQIRLQAEAFQARLKSWFEPLVEDMQRQWAGLVEKVQAAVGTSAAPVPSDNH

SEQ ID NO: 81 - protein, 121 aa, synthetic construct
FIGITELKKGGSRAATVGSLAGQPLQERAQAWGERLRARMEEMGSRTRDRLDEVKEQVAEVRAKLEEQAQQIRLQAEAFQARLKSWFEPLVEDMQRQWAGLVEKVQAAVGTSAAPVPSDNH

SEQ ID NO: 82 - protein, 121 aa, synthetic construct
FIGITELKKAAARAATVGSLAGQPLQERAQAWGERLRARMEEMGSRTRDRLDEVKEQVAEVRAKLEEQAQQIRLQAEAFQARLKSWFEPLVEDMQRQWAGLVEKVQAAVGTSAAPVPSDNH

SEQ ID NO: 83 - protein, 121 aa, synthetic construct
FIGITELKKAAYRAATVGSLAGQPLQERAQAWGERLRARMEEMGSRTRDRLDEVKEQVAEVRAKLEEQAQQIRLQAEAFQARLKSWFEPLVEDMQRQWAGLVEKVQAAVGTSAAPVPSDNH

SEQ ID NO: 84 - protein, 118 aa, synthetic construct
FIGITELLKRAATVGSLAGQPLQERAQAWGERLRARMEEMGSRTRDRLDEVKEQVAEVRAKLEEQAQQIRLQAEAFQARLKSWFEPLVEDMQRQWAGLVEKVQAAVGTSAAPVPSDNH

SEQ ID NO: 85 - protein, 123 aa, synthetic construct
FIGITELLKGGGGSRAATVGSLAGQPLQERAQAWGERLRARMEEMGSRTRDRLDEVKEQVAEVRAKLEEQAQQIRLQAEAFQARLKSWFEPLVEDMQRQWAGLVEKVQAAVGTSAAPVPSDNH

SEQ ID NO: 86 - protein, 128 aa, synthetic construct
FIGITELLKGGGGSGGGGSRAATVGSLAGQPLQERAQAWGERLRARMEEMGSRTRDRLDEVKEQVAEVRAKLEEQAQQIRLQAEAFQARLKSWFEPLVEDMQRQWAGLVEKVQAAVGTSAAPVPSDNH

SEQ ID NO: 87 - protein, 133 aa, synthetic construct
FIGITELLKGGGGSGGGGSGGGGSRAATVGSLAGQPLQERAQAWGERLRARMEEMGSRTRDRLDEVKEQVAEVRAKLEEQAQQIRLQAEAFQARLKSWFEPLVEDMQRQWAGLVEKVQAAVGTSAAPVPSDNH

SEQ ID NO: 88 - protein, 123 aa, synthetic construct
FIGITELLKEAAAKRAATVGSLAGQPLQERAQAWGERLRARMEEMGSRTRDRLDEVKEQVAEVRAKLEEQAQQIRLQAEAFQARLKSWFEPLVEDMQRQWAGLVEKVQAAVGTSAAPVPSDNH

SEQ ID NO: 89 - protein, 128 aa, synthetic construct
FIGITELLKEAAAKEAAAKRAATVGSLAGQPLQERAQAWGERLRARMEEMGSRTRDRLDEVKEQVAEVRAKLEEQAQQIRLQAEAFQARLKSWFEPLVEDMQRQWAGLVEKVQAAVGTSAAPVPSDNH

SEQ ID NO: 90 - protein, 133 aa, synthetic construct
FIGITELLKEAAAKEAAAKEAAAKRAATVGSLAGQPLQERAQAWGERLRARMEEMGSRTRDRLDEVKEQVAEVRAKLEEQAQQIRLQAEAFQARLKSWFEPLVEDMQRQWAGLVEKVQAAVGTSAAPVPSDNH

SEQ ID NO: 91 - protein, 121 aa, synthetic construct
FIGITELLKGGSRAATVGSLAGQPLQERAQAWGERLRARMEEMGSRTRDRLDEVKEQVAEVRAKLEEQAQQIRLQAEAFQARLKSWFEPLVEDMQRQWAGLVEKVQAAVGTSAAPVPSDNH

SEQ ID NO: 92 - protein, 121 aa, synthetic construct
FIGITELLKAAARAATVGSLAGQPLQERAQAWGERLRARMEEMGSRTRDRLDEVKEQVAEVRAKLEEQAQQIRLQAEAFQARLKSWFEPLVEDMQRQWAGLVEKVQAAVGTSAAPVPSDNH

SEQ ID NO: 93 - protein, 121 aa, synthetic construct
FIGITELLKAAYRAATVGSLAGQPLQERAQAWGERLRARMEEMGSRTRDRLDEVKEQVAEVRAKLEEQAQQIRLQAEAFQARLKSWFEPLVEDMQRQWAGLVEKVQAAVGTSAAPVPSDNH

SEQ ID NO: 94 - protein, 118 aa, synthetic construct
FIGITELHKRAATVGSLAGQPLQERAQAWGERLRARMEEMGSRTRDRLDEVKEQVAEVRAKLEEQAQQIRLQAEAFQARLKSWFEPLVEDMQRQWAGLVEKVQAAVGTSAAPVPSDNH

SEQ ID NO: 95 - protein, 123 aa, synthetic construct
FIGITELHKGGGGSRAATVGSLAGQPLQERAQAWGERLRARMEEMGSRTRDRLDEVKEQVAEVRAKLEEQAQQIRLQAEAFQARLKSWFEPLVEDMQRQWAGLVEKVQAAVGTSAAPVPSDNH

SEQ ID NO: 96 - protein, 128 aa, synthetic construct
FIGITELHKGGGGSGGGGSRAATVGSLAGQPLQERAQAWGERLRARMEEMGSRTRDRLDEVKEQVAEVRAKLEEQAQQIRLQAEAFQARLKSWFEPLVEDMQRQWAGLVEKVQAAVGTSAAPVPSDNH

SEQ ID NO: 97 - protein, 133 aa, synthetic construct
FIGITELHKGGGGSGGGGSGGGGSRAATVGSLAGQPLQERAQAWGERLRARMEEMGSRTRDRLDEVKEQVAEVRAKLEEQAQQIRLQAEAFQARLKSWFEPLVEDMQRQWAGLVEKVQAAVGTSAAPVPSDNH

SEQ ID NO: 98 - protein, 123 aa, synthetic construct
FIGITELHKEAAAKRAATVGSLAGQPLQERAQAWGERLRARMEEMGSRTRDRLDEVKEQVAEVRAKLEEQAQQIRLQAEAFQARLKSWFEPLVEDMQRQWAGLVEKVQAAVGTSAAPVPSDNH

SEQ ID NO: 99 - protein, 128 aa, synthetic construct
FIGITELHKEAAAKEAAAKRAATVGSLAGQPLQERAQAWGERLRARMEEMGSRTRDRLDEVKEQVAEVRAKLEEQAQQIRLQAEAFQARLKSWFEPLVEDMQRQWAGLVEKVQAAVGTSAAPVPSDNH

SEQ ID NO: 100 - protein, 133 aa, synthetic construct
FIGITELHKEAAAKEAAAKEAAAKRAATVGSLAGQPLQERAQAWGERLRARMEEMGSRTRDRLDEVKEQVAEVRAKLEEQAQQIRLQAEAFQARLKSWFEPLVEDMQRQWAGLVEKVQAAVGTSAAPVPSDNH

SEQ ID NO: 101 - protein, 121 aa, synthetic construct
FIGITELHKGGSRAATVGSLAGQPLQERAQAWGERLRARMEEMGSRTRDRLDEVKEQVAEVRAKLEEQAQQIRLQAEAFQARLKSWFEPLVEDMQRQWAGLVEKVQAAVGTSAAPVPSDNH

SEQ ID NO: 102 - protein, 121 aa, synthetic construct
FIGITELHKAAARAATVGSLAGQPLQERAQAWGERLRARMEEMGSRTRDRLDEVKEQVAEVRAKLEEQAQQIRLQAEAFQARLKSWFEPLVEDMQRQWAGLVEKVQAAVGTSAAPVPSDNH

SEQ ID NO: 103 - protein, 121 aa, synthetic construct
FIGITELHKAAYRAATVGSLAGQPLQERAQAWGERLRARMEEMGSRTRDRLDEVKEQVAEVRAKLEEQAQQIRLQAEAFQARLKSWFEPLVEDMQRQWAGLVEKVQAAVGTSAAPVPSDNH

SEQ ID NO: 104-114 - skipped (11 entries)

SEQ ID NO: 115 - protein, 145 aa, synthetic construct
FIGITELKKAGAREGAERGLSAIRERLGPLVEQGRVRAATVGSLAGQPLQERAQAWGERLRARMEEMGSRTRDRLDEVKEQVAEVRAKLEEQAQQIRLQAEAFQARLKSWFEPLVEDMQRQWAGLVEKVQAAVGTSAAPVPSDNH

SEQ ID NO: 116 - protein, 150 aa, synthetic construct
FIGITELKKGGGGSAGAREGAERGLSAIRERLGPLVEQGRVRAATVGSLAGQPLQERAQAWGERLRARMEEMGSRTRDRLDEVKEQVAEVRAKLEEQAQQIRLQAEAFQARLKSWFEPLVEDMQRQWAGLVEKVQAAVGTSAAPVPSDNH

SEQ ID NO: 117 - protein, 155 aa, synthetic construct
FIGITELKKGGGGSGGGGSAGAREGAERGLSAIRERLGPLVEQGRVRAATVGSLAGQPLQERAQAWGERLRARMEEMGSRTRDRLDEVKEQVAEVRAKLEEQAQQIRLQAEAFQARLKSWFEPLVEDMQRQWAGLVEKVQAAVGTSAAPVPSDNH

SEQ ID NO: 118 - protein, 160 aa, synthetic construct
FIGITELKKGGGGSGGGGSGGGGSAGAREGAERGLSAIRERLGPLVEQGRVRAATVGSLAGQPLQERAQAWGERLRARMEEMGSRTRDRLDEVKEQVAEVRAKLEEQAQQIRLQAEAFQARLKSWFEPLVEDMQRQWAGLVEKVQAAVGTSAAPVPSDNH

SEQ ID NO: 119 - protein, 150 aa, synthetic construct
FIGITELKKEAAAKAGAREGAERGLSAIRERLGPLVEQGRVRAATVGSLAGQPLQERAQAWGERLRARMEEMGSRTRDRLDEVKEQVAEVRAKLEEQAQQIRLQAEAFQARLKSWFEPLVEDMQRQWAGLVEKVQAAVGTSAAPVPSDNH

SEQ ID NO: 120 - protein, 155 aa, synthetic construct
FIGITELKKEAAAKEAAAKAGAREGAERGLSAIRERLGPLVEQGRVRAATVGSLAGQPLQERAQAWGERLRARMEEMGSRTRDRLDEVKEQVAEVRAKLEEQAQQIRLQAEAFQARLKSWFEPLVEDMQRQWAGLVEKVQAAVGTSAAPVPSDNH

SEQ ID NO: 121 - protein, 160 aa, synthetic construct
FIGITELKKEAAAKEAAAKEAAAKAGAREGAERGLSAIRERLGPLVEQGRVRAATVGSLAGQPLQERAQAWGERLRARMEEMGSRTRDRLDEVKEQVAEVRAKLEEQAQQIRLQAEAFQARLKSWFEPLVEDMQRQWAGLVEKVQAAVGTSAAPVPSDNH

SEQ ID NO: 122 - protein, 148 aa, synthetic construct
FIGITELKKGGSAGAREGAERGLSAIRERLGPLVEQGRVRAATVGSLAGQPLQERAQAWGERLRARMEEMGSRTRDRLDEVKEQVAEVRAKLEEQAQQIRLQAEAFQARLKSWFEPLVEDMQRQWAGLVEKVQAAVGTSAAPVPSDNH

SEQ ID NO: 123 - protein, 148 aa, synthetic construct
FIGITELKKAAAAGAREGAERGLSAIRERLGPLVEQGRVRAATVGSLAGQPLQERAQAWGERLRARMEEMGSRTRDRLDEVKEQVAEVRAKLEEQAQQIRLQAEAFQARLKSWFEPLVEDMQRQWAGLVEKVQAAVGTSAAPVPSDNH

SEQ ID NO: 124 - protein, 148 aa, synthetic construct
FIGITELKKAAYAGAREGAERGLSAIRERLGPLVEQGRVRAATVGSLAGQPLQERAQAWGERLRARMEEMGSRTRDRLDEVKEQVAEVRAKLEEQAQQIRLQAEAFQARLKSWFEPLVEDMQRQWAGLVEKVQAAVGTSAAPVPSDNH

SEQ ID NO: 125 - protein, 145 aa, synthetic construct
FIGITELLKAGAREGAERGLSAIRERLGPLVEQGRVRAATVGSLAGQPLQERAQAWGERLRARMEEMGSRTRDRLDEVKEQVAEVRAKLEEQAQQIRLQAEAFQARLKSWFEPLVEDMQRQWAGLVEKVQAAVGTSAAPVPSDNH

SEQ ID NO: 126 - protein, 150 aa, synthetic construct
FIGITELLKGGGGSAGAREGAERGLSAIRERLGPLVEQGRVRAATVGSLAGQPLQERAQAWGERLRARMEEMGSRTRDRLDEVKEQVAEVRAKLEEQAQQIRLQAEAFQARLKSWFEPLVEDMQRQWAGLVEKVQAAVGTSAAPVPSDNH

SEQ ID NO: 127 - protein, 155 aa, synthetic construct
FIGITELLKGGGGSGGGGSAGAREGAERGLSAIRERLGPLVEQGRVRAATVGSLAGQPLQERAQAWGERLRARMEEMGSRTRDRLDEVKEQVAEVRAKLEEQAQQIRLQAEAFQARLKSWFEPLVEDMQRQWAGLVEKVQAAVGTSAAPVPSDNH

SEQ ID NO: 128 - protein, 160 aa, synthetic construct
FIGITELLKGGGGSGGGGSGGGGSAGAREGAERGLSAIRERLGPLVEQGRVRAATVGSLAGQPLQERAQAWGERLRARMEEMGSRTRDRLDEVKEQVAEVRAKLEEQAQQIRLQAEAFQARLKSWFEPLVEDMQRQWAGLVEKVQAAVGTSAAPVPSDNH

SEQ ID NO: 129 - protein, 150 aa, synthetic construct
FIGITELLKEAAAKAGAREGAERGLSAIRERLGPLVEQGRVRAATVGSLAGQPLQERAQAWGERLRARMEEMGSRTRDRLDEVKEQVAEVRAKLEEQAQQIRLQAEAFQARLKSWFEPLVEDMQRQWAGLVEKVQAAVGTSAAPVPSDNH

SEQ ID NO: 130 - protein, 155 aa, synthetic construct
FIGITELLKEAAAKEAAAKAGAREGAERGLSAIRERLGPLVEQGRVRAATVGSLAGQPLQERAQAWGERLRARMEEMGSRTRDRLDEVKEQVAEVRAKLEEQAQQIRLQAEAFQARLKSWFEPLVEDMQRQWAGLVEKVQAAVGTSAAPVPSDNH

SEQ ID NO: 131 - protein, 160 aa, synthetic construct
FIGITELLKEAAAKEAAAKEAAAKAGAREGAERGLSAIRERLGPLVEQGRVRAATVGSLAGQPLQERAQAWGERLRARMEEMGSRTRDRLDEVKEQVAEVRAKLEEQAQQIRLQAEAFQARLKSWFEPLVEDMQRQWAGLVEKVQAAVGTSAAPVPSDNH

SEQ ID NO: 132 - protein, 148 aa, synthetic construct
FIGITELLKGGSAGAREGAERGLSAIRERLGPLVEQGRVRAATVGSLAGQPLQERAQAWGERLRARMEEMGSRTRDRLDEVKEQVAEVRAKLEEQAQQIRLQAEAFQARLKSWFEPLVEDMQRQWAGLVEKVQAAVGTSAAPVPSDNH

SEQ ID NO: 133 - protein, 148 aa, synthetic construct
FIGITELLKAAAAGAREGAERGLSAIRERLGPLVEQGRVRAATVGSLAGQPLQERAQAWGERLRARMEEMGSRTRDRLDEVKEQVAEVRAKLEEQAQQIRLQAEAFQARLKSWFEPLVEDMQRQWAGLVEKVQAAVGTSAAPVPSDNH

SEQ ID NO: 134 - protein, 148 aa, synthetic construct
FIGITELLKAAYAGAREGAERGLSAIRERLGPLVEQGRVRAATVGSLAGQPLQERAQAWGERLRARMEEMGSRTRDRLDEVKEQVAEVRAKLEEQAQQIRLQAEAFQARLKSWFEPLVEDMQRQWAGLVEKVQAAVGTSAAPVPSDNH

SEQ ID NO: 135 - protein, 145 aa, synthetic construct
FIGITELHKAGAREGAERGLSAIRERLGPLVEQGRVRAATVGSLAGQPLQERAQAWGERLRARMEEMGSRTRDRLDEVKEQVAEVRAKLEEQAQQIRLQAEAFQARLKSWFEPLVEDMQRQWAGLVEKVQAAVGTSAAPVPSDNH

SEQ ID NO: 136 - protein, 150 aa, synthetic construct
FIGITELHKGGGGSAGAREGAERGLSAIRERLGPLVEQGRVRAATVGSLAGQPLQERAQAWGERLRARMEEMGSRTRDRLDEVKEQVAEVRAKLEEQAQQIRLQAEAFQARLKSWFEPLVEDMQRQWAGLVEKVQAAVGTSAAPVPSDNH

SEQ ID NO: 137 - protein, 163 aa, synthetic construct
FIGITELHKGGGGSGGGGSAGAREGAERGLSAIRERLGPLVEQGRVRAATVGSLAGQPLQERAQAWGERLRARMEEMGSRTRDRLDEVKEQVAEVRAKLEEQAQQIRLQAEAFQARLKSWFEPLVEDMQRQWAGLVEKVQAAVGTSAAPVPSDNHAPVPSDNH

SEQ ID NO: 138 - protein, 160 aa, synthetic construct
FIGITELHKGGGGSGGGGSGGGGSAGAREGAERGLSAIRERLGPLVEQGRVRAATVGSLAGQPLQERAQAWGERLRARMEEMGSRTRDRLDEVKEQVAEVRAKLEEQAQQIRLQAEAFQARLKSWFEPLVEDMQRQWAGLVEKVQAAVGTSAAPVPSDNH

SEQ ID NO: 139 - protein, 150 aa, synthetic construct
FIGITELHKEAAAKAGAREGAERGLSAIRERLGPLVEQGRVRAATVGSLAGQPLQERAQAWGERLRARMEEMGSRTRDRLDEVKEQVAEVRAKLEEQAQQIRLQAEAFQARLKSWFEPLVEDMQRQWAGLVEKVQAAVGTSAAPVPSDNH

SEQ ID NO: 140 - protein, 155 aa, synthetic construct
FIGITELHKEAAAKEAAAKAGAREGAERGLSAIRERLGPLVEQGRVRAATVGSLAGQPLQERAQAWGERLRARMEEMGSRTRDRLDEVKEQVAEVRAKLEEQAQQIRLQAEAFQARLKSWFEPLVEDMQRQWAGLVEKVQAAVGTSAAPVPSDNH

SEQ ID NO: 141 - protein, 160 aa, synthetic construct
FIGITELHKEAAAKEAAAKEAAAKAGAREGAERGLSAIRERLGPLVEQGRVRAATVGSLAGQPLQERAQAWGERLRARMEEMGSRTRDRLDEVKEQVAEVRAKLEEQAQQIRLQAEAFQARLKSWFEPLVEDMQRQWAGLVEKVQAAVGTSAAPVPSDNH

SEQ ID NO: 142 - protein, 148 aa, synthetic construct
FIGITELHKGGSAGAREGAERGLSAIRERLGPLVEQGRVRAATVGSLAGQPLQERAQAWGERLRARMEEMGSRTRDRLDEVKEQVAEVRAKLEEQAQQIRLQAEAFQARLKSWFEPLVEDMQRQWAGLVEKVQAAVGTSAAPVPSDNH

SEQ ID NO: 143 - protein, 148 aa, synthetic construct
FIGITELHKAAAAGAREGAERGLSAIRERLGPLVEQGRVRAATVGSLAGQPLQERAQAWGERLRARMEEMGSRTRDRLDEVKEQVAEVRAKLEEQAQQIRLQAEAFQARLKSWFEPLVEDMQRQWAGLVEKVQAAVGTSAAPVPSDNH

SEQ ID NO: 144 - protein, 148 aa, synthetic construct
FIGITELHKAAYAGAREGAERGLSAIRERLGPLVEQGRVRAATVGSLAGQPLQERAQAWGERLRARMEEMGSRTRDRLDEVKEQVAEVRAKLEEQAQQIRLQAEAFQARLKSWFEPLVEDMQRQWAGLVEKVQAAVGTSAAPVPSDNH

SEQ ID NO: 145-155 - skipped (11 entries)

SEQ ID NO: 156 - protein, 265 aa, synthetic construct
FIGITELKKSEQVQEELLSSQVTQELRALMDETMKELKAYKSELEEQLTPVAEETRARLSKELQAAQARLGADMEDVCGRLVQYRGEVQAMLGQSTEELRVSLASHLRKLRKRLLRDADDLQKCLAVYQAGAREGAERGLSAIRERLGPLVEQGRVRAATVGSLAGQPLQERAQAWGERLRARMEEMGSRTRDRLDEVKEQVAEVRAKLEEQAQQIRLQAEAFQARLKSWFEPLVEDMQRQWAGLVEKVQAAVGTSAAPVPSDNH

SEQ ID NO: 157 - protein, 270 aa, synthetic construct
FIGITELKKGGGGSSEQVQEELLSSQVTQELRALMDETMKELKAYKSELEEQLTPVAEETRARLSKELQAAQARLGADMEDVCGRLVQYRGEVQAMLGQSTEELRVSLASHLRKLRKRLLRDADDLQKCLAVYQAGAREGAERGLSAIRERLGPLVEQGRVRAATVGSLAGQPLQERAQAWGERLRARMEEMGSRTRDRLDEVKEQVAEVRAKLEEQAQQIRLQAEAFQARLKSWFEPLVEDMQRQWAGLVEKVQAAVGTSAAPVPSDNH

SEQ ID NO: 158 - protein, 275 aa, synthetic construct
FIGITELKKGGGGSGGGGSSEQVQEELLSSQVTQELRALMDETMKELKAYKSELEEQLTPVAEETRARLSKELQAAQARLGADMEDVCGRLVQYRGEVQAMLGQSTEELRVSLASHLRKLRKRLLRDADDLQKCLAVYQAGAREGAERGLSAIRERLGPLVEQGRVRAATVGSLAGQPLQERAQAWGERLRARMEEMGSRTRDRLDEVKEQVAEVRAKLEEQAQQIRLQAEAFQARLKSWFEPLVEDMQRQWAGLVEKVQAAVGTSAAPVPSDNH

SEQ ID NO: 159 - protein, 280 aa, synthetic construct
FIGITELKKGGGGSGGGGSGGGGSSEQVQEELLSSQVTQELRALMDETMKELKAYKSELEEQLTPVAEETRARLSKELQAAQARLGADMEDVCGRLVQYRGEVQAMLGQSTEELRVSLASHLRKLRKRLLRDADDLQKCLAVYQAGAREGAERGLSAIRERLGPLVEQGRVRAATVGSLAGQPLQERAQAWGERLRARMEEMGSRTRDRLDEVKEQVAEVRAKLEEQAQQIRLQAEAFQARLKSWFEPLVEDMQRQWAGLVEKVQAAVGTSAAPVPSDNH

SEQ ID NO: 160 - protein, 270 aa, synthetic construct
FIGITELKKEAAAKSEQVQEELLSSQVTQELRALMDETMKELKAYKSELEEQLTPVAEETRARLSKELQAAQARLGADMEDVCGRLVQYRGEVQAMLGQSTEELRVSLASHLRKLRKRLLRDADDLQKCLAVYQAGAREGAERGLSAIRERLGPLVEQGRVRAATVGSLAGQPLQERAQAWGERLRARMEEMGSRTRDRLDEVKEQVAEVRAKLEEQAQQIRLQAEAFQARLKSWFEPLVEDMQRQWAGLVEKVQAAVGTSAAPVPSDNH

SEQ ID NO: 161 - protein, 275 aa, synthetic construct
FIGITELKKEAAAKEAAAKSEQVQEELLSSQVTQELRALMDETMKELKAYKSELEEQLTPVAEETRARLSKELQAAQARLGADMEDVCGRLVQYRGEVQAMLGQSTEELRVSLASHLRKLRKRLLRDADDLQKCLAVYQAGAREGAERGLSAIRERLGPLVEQGRVRAATVGSLAGQPLQERAQAWGERLRARMEEMGSRTRDRLDEVKEQVAEVRAKLEEQAQQIRLQAEAFQARLKSWFEPLVEDMQRQWAGLVEKVQAAVGTSAAPVPSDNH

SEQ ID NO: 162 - protein, 280 aa, synthetic construct
FIGITELKKEAAAKEAAAKEAAAKSEQVQEELLSSQVTQELRALMDETMKELKAYKSELEEQLTPVAEETRARLSKELQAAQARLGADMEDVCGRLVQYRGEVQAMLGQSTEELRVSLASHLRKLRKRLLRDADDLQKCLAVYQAGAREGAERGLSAIRERLGPLVEQGRVRAATVGSLAGQPLQERAQAWGERLRARMEEMGSRTRDRLDEVKEQVAEVRAKLEEQAQQIRLQAEAFQARLKSWFEPLVEDMQRQWAGLVEKVQAAVGTSAAPVPSDNH

SEQ ID NO: 163 - protein, 268 aa, synthetic construct
FIGITELKKGGSSEQVQEELLSSQVTQELRALMDETMKELKAYKSELEEQLTPVAEETRARLSKELQAAQARLGADMEDVCGRLVQYRGEVQAMLGQSTEELRVSLASHLRKLRKRLLRDADDLQKCLAVYQAGAREGAERGLSAIRERLGPLVEQGRVRAATVGSLAGQPLQERAQAWGERLRARMEEMGSRTRDRLDEVKEQVAEVRAKLEEQAQQIRLQAEAFQARLKSWFEPLVEDMQRQWAGLVEKVQAAVGTSAAPVPSDNH

SEQ ID NO: 164 - protein, 268 aa, synthetic construct
FIGITELKKAAASEQVQEELLSSQVTQELRALMDETMKELKAYKSELEEQLTPVAEETRARLSKELQAAQARLGADMEDVCGRLVQYRGEVQAMLGQSTEELRVSLASHLRKLRKRLLRDADDLQKCLAVYQAGAREGAERGLSAIRERLGPLVEQGRVRAATVGSLAGQPLQERAQAWGERLRARMEEMGSRTRDRLDEVKEQVAEVRAKLEEQAQQIRLQAEAFQARLKSWFEPLVEDMQRQWAGLVEKVQAAVGTSAAPVPSDNH

SEQ ID NO: 165 - protein, 268 aa, synthetic construct
FIGITELKKAAYSEQVQEELLSSQVTQELRALMDETMKELKAYKSELEEQLTPVAEETRARLSKELQAAQARLGADMEDVCGRLVQYRGEVQAMLGQSTEELRVSLASHLRKLRKRLLRDADDLQKCLAVYQAGAREGAERGLSAIRERLGPLVEQGRVRAATVGSLAGQPLQERAQAWGERLRARMEEMGSRTRDRLDEVKEQVAEVRAKLEEQAQQIRLQAEAFQARLKSWFEPLVEDMQRQWAGLVEKVQAAVGTSAAPVPSDNH

SEQ ID NO: 166 - protein, 265 aa, synthetic construct
FIGITELLKSEQVQEELLSSQVTQELRALMDETMKELKAYKSELEEQLTPVAEETRARLSKELQAAQARLGADMEDVCGRLVQYRGEVQAMLGQSTEELRVSLASHLRKLRKRLLRDADDLQKCLAVYQAGAREGAERGLSAIRERLGPLVEQGRVRAATVGSLAGQPLQERAQAWGERLRARMEEMGSRTRDRLDEVKEQVAEVRAKLEEQAQQIRLQAEAFQARLKSWFEPLVEDMQRQWAGLVEKVQAAVGTSAAPVPSDNH

SEQ ID NO: 167 - protein, 270 aa, synthetic construct
FIGITELLKGGGGSSEQVQEELLSSQVTQELRALMDETMKELKAYKSELEEQLTPVAEETRARLSKELQAAQARLGADMEDVCGRLVQYRGEVQAMLGQSTEELRVSLASHLRKLRKRLLRDADDLQKCLAVYQAGAREGAERGLSAIRERLGPLVEQGRVRAATVGSLAGQPLQERAQAWGERLRARMEEMGSRTRDRLDEVKEQVAEVRAKLEEQAQQIRLQAEAFQARLKSWFEPLVEDMQRQWAGLVEKVQAAVGTSAAPVPSDNH

SEQ ID NO: 168 - protein, 275 aa, synthetic construct
FIGITELLKGGGGSGGGGSSEQVQEELLSSQVTQELRALMDETMKELKAYKSELEEQLTPVAEETRARLSKELQAAQARLGADMEDVCGRLVQYRGEVQAMLGQSTEELRVSLASHLRKLRKRLLRDADDLQKCLAVYQAGAREGAERGLSAIRERLGPLVEQGRVRAATVGSLAGQPLQERAQAWGERLRARMEEMGSRTRDRLDEVKEQVAEVRAKLEEQAQQIRLQAEAFQARLKSWFEPLVEDMQRQWAGLVEKVQAAVGTSAAPVPSDNH

SEQ ID NO: 169 - protein, 280 aa, synthetic construct
FIGITELLKGGGGSGGGGSGGGGSSEQVQEELLSSQVTQELRALMDETMKELKAYKSELEEQLTPVAEETRARLSKELQAAQARLGADMEDVCGRLVQYRGEVQAMLGQSTEELRVSLASHLRKLRKRLLRDADDLQKCLAVYQAGAREGAERGLSAIRERLGPLVEQGRVRAATVGSLAGQPLQERAQAWGERLRARMEEMGSRTRDRLDEVKEQVAEVRAKLEEQAQQIRLQAEAFQARLKSWFEPLVEDMQRQWAGLVEKVQAAVGTSAAPVPSDNH

SEQ ID NO: 170 - protein, 270 aa, synthetic construct
FIGITELLKEAAAKSEQVQEELLSSQVTQELRALMDETMKELKAYKSELEEQLTPVAEETRARLSKELQAAQARLGADMEDVCGRLVQYRGEVQAMLGQSTEELRVSLASHLRKLRKRLLRDADDLQKCLAVYQAGAREGAERGLSAIRERLGPLVEQGRVRAATVGSLAGQPLQERAQAWGERLRARMEEMGSRTRDRLDEVKEQVAEVRAKLEEQAQQIRLQAEAFQARLKSWFEPLVEDMQRQWAGLVEKVQAAVGTSAAPVPSDNH

SEQ ID NO: 171 - protein, 275 aa, synthetic construct
FIGITELLKEAAAKEAAAKSEQVQEELLSSQVTQELRALMDETMKELKAYKSELEEQLTPVAEETRARLSKELQAAQARLGADMEDVCGRLVQYRGEVQAMLGQSTEELRVSLASHLRKLRKRLLRDADDLQKCLAVYQAGAREGAERGLSAIRERLGPLVEQGRVRAATVGSLAGQPLQERAQAWGERLRARMEEMGSRTRDRLDEVKEQVAEVRAKLEEQAQQIRLQAEAFQARLKSWFEPLVEDMQRQWAGLVEKVQAAVGTSAAPVPSDNH

SEQ ID NO: 172 - protein, 280 aa, synthetic construct
FIGITELLKEAAAKEAAAKEAAAKSEQVQEELLSSQVTQELRALMDETMKELKAYKSELEEQLTPVAEETRARLSKELQAAQARLGADMEDVCGRLVQYRGEVQAMLGQSTEELRVSLASHLRKLRKRLLRDADDLQKCLAVYQAGAREGAERGLSAIRERLGPLVEQGRVRAATVGSLAGQPLQERAQAWGERLRARMEEMGSRTRDRLDEVKEQVAEVRAKLEEQAQQIRLQAEAFQARLKSWFEPLVEDMQRQWAGLVEKVQAAVGTSAAPVPSDNH

SEQ ID NO: 173 - protein, 268 aa, synthetic construct
FIGITELLKGGSSEQVQEELLSSQVTQELRALMDETMKELKAYKSELEEQLTPVAEETRARLSKELQAAQARLGADMEDVCGRLVQYRGEVQAMLGQSTEELRVSLASHLRKLRKRLLRDADDLQKCLAVYQAGAREGAERGLSAIRERLGPLVEQGRVRAATVGSLAGQPLQERAQAWGERLRARMEEMGSRTRDRLDEVKEQVAEVRAKLEEQAQQIRLQAEAFQARLKSWFEPLVEDMQRQWAGLVEKVQAAVGTSAAPVPSDNH

SEQ ID NO: 174 - protein, 268 aa, synthetic construct
FIGITELLKAAASEQVQEELLSSQVTQELRALMDETMKELKAYKSELEEQLTPVAEETRARLSKELQAAQARLGADMEDVCGRLVQYRGEVQAMLGQSTEELRVSLASHLRKLRKRLLRDADDLQKCLAVYQAGAREGAERGLSAIRERLGPLVEQGRVRAATVGSLAGQPLQERAQAWGERLRARMEEMGSRTRDRLDEVKEQVAEVRAKLEEQAQQIRLQAEAFQARLKSWFEPLVEDMQRQWAGLVEKVQAAVGTSAAPVPSDNH

SEQ ID NO: 175 - protein, 268 aa, synthetic construct
FIGITELLKAAYSEQVQEELLSSQVTQELRALMDETMKELKAYKSELEEQLTPVAEETRARLSKELQAAQARLGADMEDVCGRLVQYRGEVQAMLGQSTEELRVSLASHLRKLRKRLLRDADDLQKCLAVYQAGAREGAERGLSAIRERLGPLVEQGRVRAATVGSLAGQPLQERAQAWGERLRARMEEMGSRTRDRLDEVKEQVAEVRAKLEEQAQQIRLQAEAFQARLKSWFEPLVEDMQRQWAGLVEKVQAAVGTSAAPVPSDNH

SEQ ID NO: 176 - protein, 265 aa, synthetic construct
FIGITELHKSEQVQEELLSSQVTQELRALMDETMKELKAYKSELEEQLTPVAEETRARLSKELQAAQARLGADMEDVCGRLVQYRGEVQAMLGQSTEELRVSLASHLRKLRKRLLRDADDLQKCLAVYQAGAREGAERGLSAIRERLGPLVEQGRVRAATVGSLAGQPLQERAQAWGERLRARMEEMGSRTRDRLDEVKEQVAEVRAKLEEQAQQIRLQAEAFQARLKSWFEPLVEDMQRQWAGLVEKVQAAVGTSAAPVPSDNH

SEQ ID NO: 177 - protein, 270 aa, synthetic construct
FIGITELHKGGGGSSEQVQEELLSSQVTQELRALMDETMKELKAYKSELEEQLTPVAEETRARLSKELQAAQARLGADMEDVCGRLVQYRGEVQAMLGQSTEELRVSLASHLRKLRKRLLRDADDLQKCLAVYQAGAREGAERGLSAIRERLGPLVEQGRVRAATVGSLAGQPLQERAQAWGERLRARMEEMGSRTRDRLDEVKEQVAEVRAKLEEQAQQIRLQAEAFQARLKSWFEPLVEDMQRQWAGLVEKVQAAVGTSAAPVPSDNH

SEQ ID NO: 178 - protein, 275 aa, synthetic construct
FIGITELHKGGGGSGGGGSSEQVQEELLSSQVTQELRALMDETMKELKAYKSELEEQLTPVAEETRARLSKELQAAQARLGADMEDVCGRLVQYRGEVQAMLGQSTEELRVSLASHLRKLRKRLLRDADDLQKCLAVYQAGAREGAERGLSAIRERLGPLVEQGRVRAATVGSLAGQPLQERAQAWGERLRARMEEMGSRTRDRLDEVKEQVAEVRAKLEEQAQQIRLQAEAFQARLKSWFEPLVEDMQRQWAGLVEKVQAAVGTSAAPVPSDNH

SEQ ID NO: 179 - protein, 280 aa, synthetic construct
FIGITELHKGGGGSGGGGSGGGGSSEQVQEELLSSQVTQELRALMDETMKELKAYKSELEEQLTPVAEETRARLSKELQAAQARLGADMEDVCGRLVQYRGEVQAMLGQSTEELRVSLASHLRKLRKRLLRDADDLQKCLAVYQAGAREGAERGLSAIRERLGPLVEQGRVRAATVGSLAGQPLQERAQAWGERLRARMEEMGSRTRDRLDEVKEQVAEVRAKLEEQAQQIRLQAEAFQARLKSWFEPLVEDMQRQWAGLVEKVQAAVGTSAAPVPSDNH

SEQ ID NO: 180 - protein, 270 aa, synthetic construct
FIGITELHKEAAAKSEQVQEELLSSQVTQELRALMDETMKELKAYKSELEEQLTPVAEETRARLSKELQAAQARLGADMEDVCGRLVQYRGEVQAMLGQSTEELRVSLASHLRKLRKRLLRDADDLQKCLAVYQAGAREGAERGLSAIRERLGPLVEQGRVRAATVGSLAGQPLQERAQAWGERLRARMEEMGSRTRDRLDEVKEQVAEVRAKLEEQAQQIRLQAEAFQARLKSWFEPLVEDMQRQWAGLVEKVQAAVGTSAAPVPSDNH

SEQ ID NO: 181 - protein, 275 aa, synthetic construct
FIGITELHKEAAAKEAAAKSEQVQEELLSSQVTQELRALMDETMKELKAYKSELEEQLTPVAEETRARLSKELQAAQARLGADMEDVCGRLVQYRGEVQAMLGQSTEELRVSLASHLRKLRKRLLRDADDLQKCLAVYQAGAREGAERGLSAIRERLGPLVEQGRVRAATVGSLAGQPLQERAQAWGERLRARMEEMGSRTRDRLDEVKEQVAEVRAKLEEQAQQIRLQAEAFQARLKSWFEPLVEDMQRQWAGLVEKVQAAVGTSAAPVPSDNH

SEQ ID NO: 182 - protein, 280 aa, synthetic construct
FIGITELHKEAAAKEAAAKEAAAKSEQVQEELLSSQVTQELRALMDETMKELKAYKSELEEQLTPVAEETRARLSKELQAAQARLGADMEDVCGRLVQYRGEVQAMLGQSTEELRVSLASHLRKLRKRLLRDADDLQKCLAVYQAGAREGAERGLSAIRERLGPLVEQGRVRAATVGSLAGQPLQERAQAWGERLRARMEEMGSRTRDRLDEVKEQVAEVRAKLEEQAQQIRLQAEAFQARLKSWFEPLVEDMQRQWAGLVEKVQAAVGTSAAPVPSDNH

SEQ ID NO: 183 - protein, 268 aa, synthetic construct
FIGITELHKGGSSEQVQEELLSSQVTQELRALMDETMKELKAYKSELEEQLTPVAEETRARLSKELQAAQARLGADMEDVCGRLVQYRGEVQAMLGQSTEELRVSLASHLRKLRKRLLRDADDLQKCLAVYQAGAREGAERGLSAIRERLGPLVEQGRVRAATVGSLAGQPLQERAQAWGERLRARMEEMGSRTRDRLDEVKEQVAEVRAKLEEQAQQIRLQAEAFQARLKSWFEPLVEDMQRQWAGLVEKVQAAVGTSAAPVPSDNH

SEQ ID NO: 184 - protein, 268 aa, synthetic construct
FIGITELHKAAASEQVQEELLSSQVTQELRALMDETMKELKAYKSELEEQLTPVAEETRARLSKELQAAQARLGADMEDVCGRLVQYRGEVQAMLGQSTEELRVSLASHLRKLRKRLLRDADDLQKCLAVYQAGAREGAERGLSAIRERLGPLVEQGRVRAATVGSLAGQPLQERAQAWGERLRARMEEMGSRTRDRLDEVKEQVAEVRAKLEEQAQQIRLQAEAFQARLKSWFEPLVEDMQRQWAGLVEKVQAAVGTSAAPVPSDNH

SEQ ID NO: 185 - protein, 268 aa, synthetic construct
FIGITELHKAAYSEQVQEELLSSQVTQELRALMDETMKELKAYKSELEEQLTPVAEETRARLSKELQAAQARLGADMEDVCGRLVQYRGEVQAMLGQSTEELRVSLASHLRKLRKRLLRDADDLQKCLAVYQAGAREGAERGLSAIRERLGPLVEQGRVRAATVGSLAGQPLQERAQAWGERLRARMEEMGSRTRDRLDEVKEQVAEVRAKLEEQAQQIRLQAEAFQARLKSWFEPLVEDMQRQWAGLVEKVQAAVGTSAAPVPSDNH

SEQ ID NO: 186-196 - skipped (11 entries)

SEQ ID NO: 197 - protein, 255 aa, synthetic construct
FIGITELKKSQVTQELRALMDETMKELKAYKSELEEQLTPVAEETRARLSKELQAAQARLGADMEDVCGRLVQYRGEVQAMLGQSTEELRVSLASHLRKLRKRLLRDADDLQKCLAVYQAGAREGAERGLSAIRERLGPLVEQGRVRAATVGSLAGQPLQERAQAWGERLRARMEEMGSRTRDRLDEVKEQVAEVRAKLEEQAQQIRLQAEAFQARLKSWFEPLVEDMQRQWAGLVEKVQAAVGTSAAPVPSDNH

SEQ ID NO: 198 - protein, 260 aa, synthetic construct
FIGITELKKGGGGSSQVTQELRALMDETMKELKAYKSELEEQLTPVAEETRARLSKELQAAQARLGADMEDVCGRLVQYRGEVQAMLGQSTEELRVSLASHLRKLRKRLLRDADDLQKCLAVYQAGAREGAERGLSAIRERLGPLVEQGRVRAATVGSLAGQPLQERAQAWGERLRARMEEMGSRTRDRLDEVKEQVAEVRAKLEEQAQQIRLQAEAFQARLKSWFEPLVEDMQRQWAGLVEKVQAAVGTSAAPVPSDNH

SEQ ID NO: 199 - protein, 265 aa, synthetic construct
FIGITELKKGGGGSGGGGSSQVTQELRALMDETMKELKAYKSELEEQLTPVAEETRARLSKELQAAQARLGADMEDVCGRLVQYRGEVQAMLGQSTEELRVSLASHLRKLRKRLLRDADDLQKCLAVYQAGAREGAERGLSAIRERLGPLVEQGRVRAATVGSLAGQPLQERAQAWGERLRARMEEMGSRTRDRLDEVKEQVAEVRAKLEEQAQQIRLQAEAFQARLKSWFEPLVEDMQRQWAGLVEKVQAAVGTSAAPVPSDNH

SEQ ID NO: 200 - protein, 270 aa, synthetic construct
FIGITELKKGGGGSGGGGSGGGGSSQVTQELRALMDETMKELKAYKSELEEQLTPVAEETRARLSKELQAAQARLGADMEDVCGRLVQYRGEVQAMLGQSTEELRVSLASHLRKLRKRLLRDADDLQKCLAVYQAGAREGAERGLSAIRERLGPLVEQGRVRAATVGSLAGQPLQERAQAWGERLRARMEEMGSRTRDRLDEVKEQVAEVRAKLEEQAQQIRLQAEAFQARLKSWFEPLVEDMQRQWAGLVEKVQAAVGTSAAPVPSDNH

SEQ ID NO: 201 - protein, 260 aa, synthetic construct
FIGITELKKEAAAKSQVTQELRALMDETMKELKAYKSELEEQLTPVAEETRARLSKELQAAQARLGADMEDVCGRLVQYRGEVQAMLGQSTEELRVSLASHLRKLRKRLLRDADDLQKCLAVYQAGAREGAERGLSAIRERLGPLVEQGRVRAATVGSLAGQPLQERAQAWGERLRARMEEMGSRTRDRLDEVKEQVAEVRAKLEEQAQQIRLQAEAFQARLKSWFEPLVEDMQRQWAGLVEKVQAAVGTSAAPVPSDNH

SEQ ID NO: 202 - protein, 265 aa, synthetic construct
FIGITELKKEAAAKEAAAKSQVTQELRALMDETMKELKAYKSELEEQLTPVAEETRARLSKELQAAQARLGADMEDVCGRLVQYRGEVQAMLGQSTEELRVSLASHLRKLRKRLLRDADDLQKCLAVYQAGAREGAERGLSAIRERLGPLVEQGRVRAATVGSLAGQPLQERAQAWGERLRARMEEMGSRTRDRLDEVKEQVAEVRAKLEEQAQQIRLQAEAFQARLKSWFEPLVEDMQRQWAGLVEKVQAAVGTSAAPVPSDNH

SEQ ID NO: 203 - protein, 270 aa, synthetic construct
FIGITELKKEAAAKEAAAKEAAAKSQVTQELRALMDETMKELKAYKSELEEQLTPVAEETRARLSKELQAAQARLGADMEDVCGRLVQYRGEVQAMLGQSTEELRVSLASHLRKLRKRLLRDADDLQKCLAVYQAGAREGAERGLSAIRERLGPLVEQGRVRAATVGSLAGQPLQERAQAWGERLRARMEEMGSRTRDRLDEVKEQVAEVRAKLEEQAQQIRLQAEAFQARLKSWFEPLVEDMQRQWAGLVEKVQAAVGTSAAPVPSDNH

SEQ ID NO: 204 - protein, 258 aa, synthetic construct
FIGITELKKGGSSQVTQELRALMDETMKELKAYKSELEEQLTPVAEETRARLSKELQAAQARLGADMEDVCGRLVQYRGEVQAMLGQSTEELRVSLASHLRKLRKRLLRDADDLQKCLAVYQAGAREGAERGLSAIRERLGPLVEQGRVRAATVGSLAGQPLQERAQAWGERLRARMEEMGSRTRDRLDEVKEQVAEVRAKLEEQAQQIRLQAEAFQARLKSWFEPLVEDMQRQWAGLVEKVQAAVGTSAAPVPSDNH

SEQ ID NO: 205 - protein, 258 aa, synthetic construct
FIGITELKKAAASQVTQELRALMDETMKELKAYKSELEEQLTPVAEETRARLSKELQAAQARLGADMEDVCGRLVQYRGEVQAMLGQSTEELRVSLASHLRKLRKRLLRDADDLQKCLAVYQAGAREGAERGLSAIRERLGPLVEQGRVRAATVGSLAGQPLQERAQAWGERLRARMEEMGSRTRDRLDEVKEQVAEVRAKLEEQAQQIRLQAEAFQARLKSWFEPLVEDMQRQWAGLVEKVQAAVGTSAAPVPSDNH

SEQ ID NO: 206 - protein, 258 aa, synthetic construct
FIGITELKKAAYSQVTQELRALMDETMKELKAYKSELEEQLTPVAEETRARLSKELQAAQARLGADMEDVCGRLVQYRGEVQAMLGQSTEELRVSLASHLRKLRKRLLRDADDLQKCLAVYQAGAREGAERGLSAIRERLGPLVEQGRVRAATVGSLAGQPLQERAQAWGERLRARMEEMGSRTRDRLDEVKEQVAEVRAKLEEQAQQIRLQAEAFQARLKSWFEPLVEDMQRQWAGLVEKVQAAVGTSAAPVPSDNH

SEQ ID NO: 207 - protein, 255 aa, synthetic construct
FIGITELLKSQVTQELRALMDETMKELKAYKSELEEQLTPVAEETRARLSKELQAAQARLGADMEDVCGRLVQYRGEVQAMLGQSTEELRVSLASHLRKLRKRLLRDADDLQKCLAVYQAGAREGAERGLSAIRERLGPLVEQGRVRAATVGSLAGQPLQERAQAWGERLRARMEEMGSRTRDRLDEVKEQVAEVRAKLEEQAQQIRLQAEAFQARLKSWFEPLVEDMQRQWAGLVEKVQAAVGTSAAPVPSDNH

SEQ ID NO: 208 - protein, 260 aa, synthetic construct
FIGITELLKGGGGSSQVTQELRALMDETMKELKAYKSELEEQLTPVAEETRARLSKELQAAQARLGADMEDVCGRLVQYRGEVQAMLGQSTEELRVSLASHLRKLRKRLLRDADDLQKCLAVYQAGAREGAERGLSAIRERLGPLVEQGRVRAATVGSLAGQPLQERAQAWGERLRARMEEMGSRTRDRLDEVKEQVAEVRAKLEEQAQQIRLQAEAFQARLKSWFEPLVEDMQRQWAGLVEKVQAAVGTSAAPVPSDNH

SEQ ID NO: 209 - protein, 265 aa, synthetic construct
FIGITELLKGGGGSGGGGSSQVTQELRALMDETMKELKAYKSELEEQLTPVAEETRARLSKELQAAQARLGADMEDVCGRLVQYRGEVQAMLGQSTEELRVSLASHLRKLRKRLLRDADDLQKCLAVYQAGAREGAERGLSAIRERLGPLVEQGRVRAATVGSLAGQPLQERAQAWGERLRARMEEMGSRTRDRLDEVKEQVAEVRAKLEEQAQQIRLQAEAFQARLKSWFEPLVEDMQRQWAGLVEKVQAAVGTSAAPVPSDNH

SEQ ID NO: 210 - protein, 270 aa, synthetic construct
FIGITELLKGGGGSGGGGSGGGGSSQVTQELRALMDETMKELKAYKSELEEQLTPVAEETRARLSKELQAAQARLGADMEDVCGRLVQYRGEVQAMLGQSTEELRVSLASHLRKLRKRLLRDADDLQKCLAVYQAGAREGAERGLSAIRERLGPLVEQGRVRAATVGSLAGQPLQERAQAWGERLRARMEEMGSRTRDRLDEVKEQVAEVRAKLEEQAQQIRLQAEAFQARLKSWFEPLVEDMQRQWAGLVEKVQAAVGTSAAPVPSDNH

SEQ ID NO: 211 - protein, 260 aa, synthetic construct
FIGITELLKEAAAKSQVTQELRALMDETMKELKAYKSELEEQLTPVAEETRARLSKELQAAQARLGADMEDVCGRLVQYRGEVQAMLGQSTEELRVSLASHLRKLRKRLLRDADDLQKCLAVYQAGAREGAERGLSAIRERLGPLVEQGRVRAATVGSLAGQPLQERAQAWGERLRARMEEMGSRTRDRLDEVKEQVAEVRAKLEEQAQQIRLQAEAFQARLKSWFEPLVEDMQRQWAGLVEKVQAAVGTSAAPVPSDNH

SEQ ID NO: 212 - protein, 265 aa, synthetic construct
FIGITELLKEAAAKEAAAKSQVTQELRALMDETMKELKAYKSELEEQLTPVAEETRARLSKELQAAQARLGADMEDVCGRLVQYRGEVQAMLGQSTEELRVSLASHLRKLRKRLLRDADDLQKCLAVYQAGAREGAERGLSAIRERLGPLVEQGRVRAATVGSLAGQPLQERAQAWGERLRARMEEMGSRTRDRLDEVKEQVAEVRAKLEEQAQQIRLQAEAFQARLKSWFEPLVEDMQRQWAGLVEKVQAAVGTSAAPVPSDNH

SEQ ID NO: 213 - protein, 270 aa, synthetic construct
FIGITELLKEAAAKEAAAKEAAAKSQVTQELRALMDETMKELKAYKSELEEQLTPVAEETRARLSKELQAAQARLGADMEDVCGRLVQYRGEVQAMLGQSTEELRVSLASHLRKLRKRLLRDADDLQKCLAVYQAGAREGAERGLSAIRERLGPLVEQGRVRAATVGSLAGQPLQERAQAWGERLRARMEEMGSRTRDRLDEVKEQVAEVRAKLEEQAQQIRLQAEAFQARLKSWFEPLVEDMQRQWAGLVEKVQAAVGTSAAPVPSDNH

SEQ ID NO: 214 - protein, 258 aa, synthetic construct
FIGITELLKGGSSQVTQELRALMDETMKELKAYKSELEEQLTPVAEETRARLSKELQAAQARLGADMEDVCGRLVQYRGEVQAMLGQSTEELRVSLASHLRKLRKRLLRDADDLQKCLAVYQAGAREGAERGLSAIRERLGPLVEQGRVRAATVGSLAGQPLQERAQAWGERLRARMEEMGSRTRDRLDEVKEQVAEVRAKLEEQAQQIRLQAEAFQARLKSWFEPLVEDMQRQWAGLVEKVQAAVGTSAAPVPSDNH

SEQ ID NO: 215 - protein, 258 aa, synthetic construct
FIGITELLKAAASQVTQELRALMDETMKELKAYKSELEEQLTPVAEETRARLSKELQAAQARLGADMEDVCGRLVQYRGEVQAMLGQSTEELRVSLASHLRKLRKRLLRDADDLQKCLAVYQAGAREGAERGLSAIRERLGPLVEQGRVRAATVGSLAGQPLQERAQAWGERLRARMEEMGSRTRDRLDEVKEQVAEVRAKLEEQAQQIRLQAEAFQARLKSWFEPLVEDMQRQWAGLVEKVQAAVGTSAAPVPSDNH

SEQ ID NO: 216 - protein, 258 aa, synthetic construct
FIGITELLKAAYSQVTQELRALMDETMKELKAYKSELEEQLTPVAEETRARLSKELQAAQARLGADMEDVCGRLVQYRGEVQAMLGQSTEELRVSLASHLRKLRKRLLRDADDLQKCLAVYQAGAREGAERGLSAIRERLGPLVEQGRVRAATVGSLAGQPLQERAQAWGERLRARMEEMGSRTRDRLDEVKEQVAEVRAKLEEQAQQIRLQAEAFQARLKSWFEPLVEDMQRQWAGLVEKVQAAVGTSAAPVPSDNH

SEQ ID NO: 217 - protein, 255 aa, synthetic construct
FIGITELHKSQVTQELRALMDETMKELKAYKSELEEQLTPVAEETRARLSKELQAAQARLGADMEDVCGRLVQYRGEVQAMLGQSTEELRVSLASHLRKLRKRLLRDADDLQKCLAVYQAGAREGAERGLSAIRERLGPLVEQGRVRAATVGSLAGQPLQERAQAWGERLRARMEEMGSRTRDRLDEVKEQVAEVRAKLEEQAQQIRLQAEAFQARLKSWFEPLVEDMQRQWAGLVEKVQAAVGTSAAPVPSDNH

SEQ ID NO: 218 - protein, 260 aa, synthetic construct
FIGITELHKGGGGSSQVTQELRALMDETMKELKAYKSELEEQLTPVAEETRARLSKELQAAQARLGADMEDVCGRLVQYRGEVQAMLGQSTEELRVSLASHLRKLRKRLLRDADDLQKCLAVYQAGAREGAERGLSAIRERLGPLVEQGRVRAATVGSLAGQPLQERAQAWGERLRARMEEMGSRTRDRLDEVKEQVAEVRAKLEEQAQQIRLQAEAFQARLKSWFEPLVEDMQRQWAGLVEKVQAAVGTSAAPVPSDNH

SEQ ID NO: 219 - protein, 265 aa, synthetic construct
FIGITELHKGGGGSGGGGSSQVTQELRALMDETMKELKAYKSELEEQLTPVAEETRARLSKELQAAQARLGADMEDVCGRLVQYRGEVQAMLGQSTEELRVSLASHLRKLRKRLLRDADDLQKCLAVYQAGAREGAERGLSAIRERLGPLVEQGRVRAATVGSLAGQPLQERAQAWGERLRARMEEMGSRTRDRLDEVKEQVAEVRAKLEEQAQQIRLQAEAFQARLKSWFEPLVEDMQRQWAGLVEKVQAAVGTSAAPVPSDNH

SEQ ID NO: 220 - protein, 270 aa, synthetic construct
FIGITELHKGGGGSGGGGSGGGGSSQVTQELRALMDETMKELKAYKSELEEQLTPVAEETRARLSKELQAAQARLGADMEDVCGRLVQYRGEVQAMLGQSTEELRVSLASHLRKLRKRLLRDADDLQKCLAVYQAGAREGAERGLSAIRERLGPLVEQGRVRAATVGSLAGQPLQERAQAWGERLRARMEEMGSRTRDRLDEVKEQVAEVRAKLEEQAQQIRLQAEAFQARLKSWFEPLVEDMQRQWAGLVEKVQAAVGTSAAPVPSDNH

SEQ ID NO: 221 - protein, 260 aa, synthetic construct
FIGITELHKEAAAKSQVTQELRALMDETMKELKAYKSELEEQLTPVAEETRARLSKELQAAQARLGADMEDVCGRLVQYRGEVQAMLGQSTEELRVSLASHLRKLRKRLLRDADDLQKCLAVYQAGAREGAERGLSAIRERLGPLVEQGRVRAATVGSLAGQPLQERAQAWGERLRARMEEMGSRTRDRLDEVKEQVAEVRAKLEEQAQQIRLQAEAFQARLKSWFEPLVEDMQRQWAGLVEKVQAAVGTSAAPVPSDNH

SEQ ID NO: 222 - protein, 265 aa, synthetic construct
FIGITELHKEAAAKEAAAKSQVTQELRALMDETMKELKAYKSELEEQLTPVAEETRARLSKELQAAQARLGADMEDVCGRLVQYRGEVQAMLGQSTEELRVSLASHLRKLRKRLLRDADDLQKCLAVYQAGAREGAERGLSAIRERLGPLVEQGRVRAATVGSLAGQPLQERAQAWGERLRARMEEMGSRTRDRLDEVKEQVAEVRAKLEEQAQQIRLQAEAFQARLKSWFEPLVEDMQRQWAGLVEKVQAAVGTSAAPVPSDNH

SEQ ID NO: 223 - protein, 270 aa, synthetic construct
FIGITELHKEAAAKEAAAKEAAAKSQVTQELRALMDETMKELKAYKSELEEQLTPVAEETRARLSKELQAAQARLGADMEDVCGRLVQYRGEVQAMLGQSTEELRVSLASHLRKLRKRLLRDADDLQKCLAVYQAGAREGAERGLSAIRERLGPLVEQGRVRAATVGSLAGQPLQERAQAWGERLRARMEEMGSRTRDRLDEVKEQVAEVRAKLEEQAQQIRLQAEAFQARLKSWFEPLVEDMQRQWAGLVEKVQAAVGTSAAPVPSDNH

SEQ ID NO: 224 - protein, 258 aa, synthetic construct
FIGITELHKGGSSQVTQELRALMDETMKELKAYKSELEEQLTPVAEETRARLSKELQAAQARLGADMEDVCGRLVQYRGEVQAMLGQSTEELRVSLASHLRKLRKRLLRDADDLQKCLAVYQAGAREGAERGLSAIRERLGPLVEQGRVRAATVGSLAGQPLQERAQAWGERLRARMEEMGSRTRDRLDEVKEQVAEVRAKLEEQAQQIRLQAEAFQARLKSWFEPLVEDMQRQWAGLVEKVQAAVGTSAAPVPSDNH

SEQ ID NO: 225 - protein, 258 aa, synthetic construct
FIGITELHKAAASQVTQELRALMDETMKELKAYKSELEEQLTPVAEETRARLSKELQAAQARLGADMEDVCGRLVQYRGEVQAMLGQSTEELRVSLASHLRKLRKRLLRDADDLQKCLAVYQAGAREGAERGLSAIRERLGPLVEQGRVRAATVGSLAGQPLQERAQAWGERLRARMEEMGSRTRDRLDEVKEQVAEVRAKLEEQAQQIRLQAEAFQARLKSWFEPLVEDMQRQWAGLVEKVQAAVGTSAAPVPSDNH

SEQ ID NO: 226 - protein, 258 aa, synthetic construct
FIGITELHKAAYSQVTQELRALMDETMKELKAYKSELEEQLTPVAEETRARLSKELQAAQARLGADMEDVCGRLVQYRGEVQAMLGQSTEELRVSLASHLRKLRKRLLRDADDLQKCLAVYQAGAREGAERGLSAIRERLGPLVEQGRVRAATVGSLAGQPLQERAQAWGERLRARMEEMGSRTRDRLDEVKEQVAEVRAKLEEQAQQIRLQAEAFQARLKSWFEPLVEDMQRQWAGLVEKVQAAVGTSAAPVPSDNH

SEQ ID NO: 227 - skipped

SEQ ID NO: 228 - protein, 45 aa, synthetic construct
FIGITELKKAAYRAHYNIVTFAAYRAHYNIVTFAAYRAHYNIVTF

SEQ ID NO: 229 - protein, 45 aa, synthetic construct
FIGITELKKAAARAHYNIVTFAAARAHYNIVTFAAARAHYNIVTF

SEQ ID NO: 230 - protein, 45 aa, synthetic construct
FIGITELKKGGSRAHYNIVTFGGSRAHYNIVTFGGSRAHYNIVTF

SEQ ID NO: 231 - protein, 43 aa, synthetic construct
GITELKKAAYRAHYNIVTFAAYRAHYNIVTFAAYRAHYNIVTF

SEQ ID NO: 232 - protein, 43 aa, synthetic construct
GITELKKAAARAHYNIVTFAAARAHYNIVTFAAARAHYNIVTF

SEQ ID NO: 233 - protein, 43 aa, synthetic construct
GITELKKGGSRAHYNIVTFGGSRAHYNIVTFGGSRAHYNIVTF

SEQ ID NO: 234 - protein, 33 aa, synthetic construct
FIGITELKKAAYRAHYNIVTFAAYRAHYNIVTF

SEQ ID NO: 235 - protein, 33 aa, synthetic construct
FIGITELKKAAARAHYNIVTFAAARAHYNIVTF

SEQ ID NO: 236 - protein, 33 aa, synthetic construct
FIGITELKKGGSRAHYNIVTFGGSRAHYNIVTF

SEQ ID NO: 237 - protein, 32 aa, synthetic construct
FIGITELKKGGSAVGALKVPRNQDWLGVPRQL

SEQ ID NO: 238 - protein, 32 aa, synthetic construct
FIGITELLKGGSAVGALKVPRNQDWLGVPRQL

SEQ ID NO: 239 - protein, 32 aa, synthetic construct
FIGITELHKGGSAVGALKVPRNQDWLGVPRQL

SEQ ID NO: 240 - protein, 40 aa, synthetic construct
FIGITELKKSSAESLKISQAVHAAHAEINEAGREVVGSAE

SEQ ID NO: 241 - protein, 40 aa, synthetic construct
FIGITELLKSSAESLKISQAVHAAHAEINEAGREVVGSAE

SEQ ID NO: 242 - protein, 40 aa, synthetic construct
FIGITELHKSSAESLKISQAVHAAHAEINEAGREVVGSAE

SEQ ID NO: 243 - protein, 43 aa, synthetic construct
FIGITELKKGGSSSAESLKISQAVHAAHAEINEAGREVVGSAE

SEQ ID NO: 244 - protein, 43 aa, synthetic construct
FIGITELLKGGSSSAESLKISQAVHAAHAEINEAGREVVGSAE

SEQ ID NO: 245 - protein, 43 aa, synthetic construct
FIGITELHKGGSSSAESLKISQAVHAAHAEINEAGREVVGSAE

SEQ ID NO: 246 - protein, 118 aa, synthetic construct
QVQLVQSGAEVKKPGASVKVSCKASGFNIKDFNIHWVRQAPGQGLEWIGRIDPESGDAEYVPKFQGRVTMTRDTSTSTVYMELSSLRSEDTAVYYCTTGSYDLDVEYWGQGTLVTVSS

SEQ ID NO: 247 - protein, 118 aa, synthetic construct
QVQLVQSGAEVKKPGASVKVSCKASGFNIKDFNIHWVRQAPGQGLEWIGRIDPEGGDAEYVPKFQGRVTMTRDTSTSTVYMELSSLRSEDTAVYYCTTGSYDLDVEYWGQGTLVTVSS

SEQ ID NO: 248 - protein, 118 aa, synthetic construct
QVQLVQSGAEVKKPGASVKVSCKASGFNIKDFNIHWVRQAPGQGLEWIGRIDPEQGDAEYVPKFQGRVTMTRDTSTSTVYMELSSLRSEDTAVYYCTTGSYDLDVEYWGQGTLVTVSS

SEQ ID NO: 249 - protein, 118 aa, synthetic construct
QVQLVQSGAEVKKPGASVKVSCKASGFNIKDFNIHWVRQAPGQGLEWIGRIDPEDGDAEYVPKFQGRVTMTRDTSTSTVYMELSSLRSEDTAVYYCTTGSYDLDVEYWGQGTLVTVSS

SEQ ID NO: 250 - protein, 118 aa, synthetic construct
QVQLVQSGAEVKKPGASVKVSCKASGFNIKDFNIHWVRQAPGQGLEWIGRIDPENADAEYVPKFQGRVTMTRDTSTSTVYMELSSLRSEDTAVYYCTTGSYDLDVEYWGQGTLVTVSS

SEQ ID NO: 251 - protein, 118 aa, synthetic construct
QVQLVQSGAEVKKPGASVKVSCKASGFNIKDFNIHWVRQAPGQGLEWIGRIDPENGDAEYVPKFQGRVTMTRDTSTSTVYMELSSLRSEDTAVYYCTTGSYDLDVEYWGQGTLVTVSS

SEQ ID NO: 252 - protein, 8 aa, synthetic construct
FNIKDFNI

SEQ ID NO: 253 - protein, 17 aa, synthetic construct
IGRIDPEXAXBDAEYVP

SEQ ID NO: 254 - protein, 10 aa, synthetic construct
TTGSYDLDVE

SEQ ID NO: 255 - protein, 107 aa, synthetic construct
DIQMTQSPSSLSASVGDRVTITCHASQNINVWLSWYQQKPGKAPKLLIYKASTLHTGVPSRFSGSGSGTDFTLTISSLQPEDFATYYCQQGQSYPLTFGQGTKLEIK

SEQ ID NO: 256 - protein, 11 aa, synthetic construct
HASQNINVWLS

SEQ ID NO: 257 - protein, 7 aa, synthetic construct
KASTLHT

SEQ ID NO: 258 - protein, 9 aa, synthetic construct
QQGQSYPLT

SEQ ID NO: 259 - protein, 6 aa, synthetic construct
QSISSY

SEQ ID NO: 260 - skipped

SEQ ID NO: 261 - protein, 9 aa, synthetic construct
QQGYPYPFT

SEQ ID NO: 262 - protein, 8 aa, synthetic construct
GFTFSSYA

SEQ ID NO: 263 - protein, 8 aa, synthetic construct
ISGYSGST

SEQ ID NO: 264 - protein, 14 aa, synthetic construct
ARYYSYYGYYYFDY

SEQ ID NO: 265 - protein, 107 aa, synthetic construct
DIQMTQSPSSLSASVGDRVTITCRASQSISSYLNWYQQKPGKAPKLLIYAASSLQSGVPSRFSGSGSGTDFTLTISSLQPEDFATYYCQQGYPYPFTFGQGTKLEIK

SEQ ID NO: 266 - protein, 121 aa, synthetic construct
EVQLLESGGGLVQPGGSLRLSCAASGFTFSSYAMSWVRQAPGKGLEWVSGISGYSGSTYYADSVKGRFTISRDNSKNTLYLQMNSLRAEDTAVYYCARYYSYYGYYYFDYWGQGTLVTVSS

SEQ ID NO: 267 - protein, 120 aa, synthetic construct [sequence omitted]

SEQ ID NO: 268 - protein, 107 aa, synthetic construct [sequence omitted]

SEQ ID NO: 269 - protein, 121 aa, synthetic construct [sequence omitted]

SEQ ID NO: 270 - protein, 106 aa, synthetic construct [sequence omitted]

SEQ ID NO: 271 - protein, 33 aa, synthetic construct
RAHYNIVTFAAYRAHYNIVTFAAYRAHYNIVTF

SEQ ID NO: 272 - protein, 33 aa, synthetic construct
RAHYNIVTFAAARAHYNIVTFAAARAHYNIVTF

SEQ ID NO: 273 - protein, 33 aa, synthetic construct
RAHYNIVTFGGSRAHYNIVTFGGSRAHYNIVTF

SEQ ID NO: 274 - protein, 21 aa, synthetic construct
RAHYNIVTFAAYRAHYNIVTF

SEQ ID NO: 275 - protein, 21 aa, synthetic construct
RAHYNIVTFAAARAHYNIVTF

SEQ ID NO: 276 - protein, 21 aa, synthetic construct
RAHYNIVTFGGSRAHYNIVTF

SEQ ID NO: 277 - protein, 20 aa, synthetic construct
AVGALKVPRNQDWLGVPRQL

SEQ ID NO: 278 - protein, 31 aa, synthetic construct
SSAESLKISQAVHAAHAEINEAGREVVGSAE

SEQ ID NO: 279 - RNA, 705 nt, synthetic construct
  source 1..705: mol_type = other RNA
atgggaagcaacagcttcagcacaagcgccttcggtccagttgccttcagcctgggcctgctgctggtgctgcctgctgccttccctgccccacaccatcaccatcaccatggagggggcggtggcggtggaggtgtcttcacactggaggacttcgttggggactggcgccagacagccggctacaacctggaccaagtcctggaacagggaggtgtgagcagcctgttccagaatctgggggtgagcgtaactccgatccaacgcattgtcctgagcggtgagaatgggctgaagatcgacatccatgtcatcatcccgtatgagggtctgagcggcgaccaaatgggccagatcgagaagatattcaaggtggtgtaccctgtggatgatcatcacttcaaggtgatcctgcactatggcacactggtaatcgacggggttacgccgaacatgatcgactacttcggacgcccgtatgaaggcatcgccgtgttcgacggcaagaagatcactgtaacagggaccctgtggaacggcaacaagattatcgacgagcgcctgatcaaccccgacggcagcctgctgttccgcgtaaccatcaacggagtgaccggctggcgcctgtgcgaacgcattctggcgggaggtggcggaggcggtggaggcgcctggcgccacccccagttcggcggctgataatag

SEQ ID NO: 280 - RNA, 1671 nt, synthetic construct
  source 1..1671: mol_type = other RNA
atggaggatgcgaaaaatataaagaaaggtccggcacctttctatcctctggaggatgggacggctggtgagcagctgcacaaagccatgaaacgctatgcactggtacctggtactatcgcttttacagatgcccacatagaggtggacatcacatacgcggagtattttgagatgagcgtccgcctggctgaggcaatgaaacgctacggcctgaatactaaccaccgcatcgtggtttgtagcgagaacagcctgcaatttttcatgcccgtactgggagcactgtttatcggggttgctgtggcccccgcgaacgatatatataatgaacgcgagctgctgaacagcatgggtataagccagccaacagtggtgtttgtcagcaagaaagggctgcagaagatactgaacgtccagaaaaaactgcctattattcaaaaaataattatcatggacagcaaaacagactatcagggttttcagagcatgtacaccttcgtaaccagccatctgcctccgggctttaatgagtatgattttgtacctgagagctttgatcgcgataaaaccatcgctctgattatgaatagcagcggaagcacgggtctgccaaaaggagtcgcactgccacaccgcacagcttgtgtacgctttagccatgcacgcgacccaattttcggtaaccagatcattcccgacacagcaatcctgagcgttgtcccttttcaccacggcttcggtatgtttaccacgctgggatatctgatatgcggattccgcgttgtactgatgtaccgcttcgaggaggaactgttcctgcgcagcctgcaagactataagattcaaagcgcgctgctggtacctactctgtttagcttcttcgcgaaaagcactctgatcgacaaatatgacctgagcaacctgcatgagatagctagcgggggtgcgcccctgagcaaagaggtaggagaggcggttgccaaacgctttcacctgcctgggattcgccagggatacgggctgacggagactaccagcgccattctgataacacctgagggtgatgacaaacccggagccgtcggcaaggttgttcctttcttcgaggctaaagttgttgatctggacaccgggaagactctgggggtcaatcagcgcggagagctgtgcgtacgcggccctatgataatgagcggttatgtcaataaccccgaggcgacgaacgccctgatcgataaagatgggtggctgcatagcggggacatagcgtattgggatgaggacgagcatttctttatagttgaccgcctgaagagcctgatcaaatacaaaggctatcaggtcgcacctgccgagctggagagcattctgctgcaacaccctaatatattcgatgccggcgtggctgggctgccagacgatgacgccggggagctgccagctgccgttgtggttctggagcacggtaaaaccatgactgaaaaggagatcgtagactatgttgctagccaggtaactacggcgaaaaaactgcgcggaggtgtggtctttgtagatgaggtgccgaaggggctgactggtaagctggatgcccgcaagatccgcgagatcctgatcaaagctaagaagggcggtaaaattgcagtacatcatcaccaccatcattaa

SEQ ID NO: 281 - RNA, 720 nt, synthetic construct
  source 1..720: mol_type = other RNA
atggtttctaagggtgaggagctgttcactggagtggtaccgattctggtagagctggatggcgacgtaaatggacacaaatttagcgtcagcggcgaaggtgagggcgacgccacatacgggaagctgacgctgaagttcatttgtacgaccggtaaactgcccgtgccgtggccgactttggtcacaaccctgacctacggcgtccagtgttttagccgctaccccgaccatatgaagcagcacgatttcttcaagagcgcaatgcctgagggatacgttcaggagcgcaccatcttttttaaagacgacggcaactataaaacccgcgcggaagtaaaattcgagggggacactctggtcaatcgcatagagctgaagggaattgatttcaaggaggatggcaacatactgggacataagctggagtataattacaatagccacaacgtttatattatggctgacaaacagaagaatggtattaaggctaactttaagatccgccacaacatcgaagatgggagcgtccaactggcagatcactatcagcagaatactcctatcggtgatgggccggttctgctgcccgataaccattacctcagcacccaaagcgcgctgagcaaggaccccaacgagaaacgcgatcatatggttctgctggagttcgtcacggctgccggtataacactgggcatggacgagctgtataaataa

SEQ ID NO: 282 - RNA, 558 nt, synthetic construct
  source 1..558: mol_type = other RNA
atgggagtcaaagttctgtttgccctgatctgcatcgctgtggccgaggccaagcccaccgagaacaacgaagacttcaacatcgtggccgtggccagcaacttcgcgaccacggatctcgatgctgaccgcgggaagttgcccggcaagaagctgccgctggaggtgctcaaagagatggaagccaatgcccggaaagctggctgcaccaggggctgtctgatctgcctgtcccacatcaagtgcacgcccaagatgaagaagttcatcccaggacgctgccacacctacgaaggcgacaaagagtccgcacagggcggcataggcgaggcgatcgtcgacattcctgagattcctgggttcaaggacttggagcccatggagcagttcatcgcacaggtcgatctgtgtgtggactgcacaactggctgcctcaaagggcttgccaacgtgcagtgttctgacctgctcaagaagtggctgccgcaacgctgtgcgacctttgccagcaagatccagggccaggtggacaagatcaagggggccggtggtgactaa

SEQ ID NO: 283 - protein, 299 aa, synthetic construct
KVEQAVETEPEPELRQQTEWQSGQRWELALGRFWDYLRWVQTLSEQVQEELLSSQVTQELRALMDETMKELKAYKSELEEQLTPVAEETRARLSKELQAAQARLGADMEDVCGRLVQYRGEVQAMLGQSTEELRVRLASHLRKLRKRLLRDADDLQKCLAVYQAGAREGAERGLSAIRERLGPLVEQGRVRAATVGSLAGQPLQERAQAWGERLRARMEEMGSRTRDRLDEVKEQVAEVRAKLEEQAQQIRLQAEAFQARLKSWFEPLVEDMQRQWAGLVEKVQAAVGTSAAPVPSDNH

SEQ ID NO: 284 - protein, 299 aa, synthetic construct
KVEQAVETEPEPELRQQTEWQSGQRWELALGRFWDYLRWVQTLSEQVQEELLSSQVTQELRALMDETMKELKAYKSELEEQLTPVAEETRARLSKELQAAQARLGADMEDVCGRLVQYRGEVQAMLGQSTEELRVRLASHLRKLRKRLLRDADDLQKRLAVYQAGAREGAERGLSAIRERLGPLVEQGRVRAATVGSLAGQPLQERAQAWGERLRARMEEMGSRTRDRLDEVKEQVAEVRAKLEEQAQQIRLQAEAFQARLKSWFEPLVEDMQRQWAGLVEKVQAAVGTSAAPVPSDNH

SEQ ID NO: 285 - protein, 299 aa, synthetic construct
KVEQAVETEPEPELRQQTEWQSGQRWELALGRFWDYLRWVQTLSEQVQEELLSSQVTQELRALMDETMKELKAYKSELEEQLTPVAEETRARLSKELQAAQARLGADMEDVRGRLVQYRGEVQAMLGQSTEELRVRLASHLRKLRKRLLRDADDLQKRLAVYQAGAREGAERGLSAIRERLGPLVEQGRVRAATVGSLAGQPLQERAQAWGERLRARMEEMGSRTRDRLDEVKEQVAEVRAKLEEQAQQIRLQAEAFQARLKSWFEPLVEDMQRQWAGLVEKVQAAVGTSAAPVPSDNH

SEQ ID NO: 286 - protein, 290 aa, synthetic construct
PEPELRQQTEWQSGQRWELALGRFWDYLRWVQTLSEQVQEELLSSQVTQELRALMDETMKELKAYKSELEEQLTPVAEETRARLSKELQAAQARLGADMEDVCGRLVQYRGEVQAMLGQSTEELRVSLASHLRKLRKRLLRDADDLQKCLAVYQAGAREGAERGLSAIRERLGPLVEQGRVRAATVGSLAGQPLQERAQAWGERLRARMEEMGSRTRDRLDEVKEQVAEVRAKLEEQAQQIRLQAEAFQARLKSWFEPLVEDMQRQWAGLVEKVQAAVGTSAAPVPSDNH

SEQ ID NO: 287 - protein, 299 aa, synthetic construct
FIGITELXKPEPELRQQTEWQSGQRWELALGRFWDYLRWVQTLSEQVQEELLSSQVTQELRALMDETMKELKAYKSELEEQLTPVAEETRARLSKELQAAQARLGADMEDVCGRLVQYRGEVQAMLGQSTEELRVSLASHLRKLRKRLLRDADDLQKCLAVYQAGAREGAERGLSAIRERLGPLVEQGRVRAATVGSLAGQPLQERAQAWGERLRARMEEMGSRTRDRLDEVKEQVAEVRAKLEEQAQQIRLQAEAFQARLKSWFEPLVEDMQRQWAGLVEKVQAAVGTSAAPVPSDNH

SEQ ID NO: 288 - protein, 304 aa, synthetic construct
FIGITELXKGGGGSPEPELRQQTEWQSGQRWELALGRFWDYLRWVQTLSEQVQEELLSSQVTQELRALMDETMKELKAYKSELEEQLTPVAEETRARLSKELQAAQARLGADMEDVCGRLVQYRGEVQAMLGQSTEELRVSLASHLRKLRKRLLRDADDLQKCLAVYQAGAREGAERGLSAIRERLGPLVEQGRVRAATVGSLAGQPLQERAQAWGERLRARMEEMGSRTRDRLDEVKEQVAEVRAKLEEQAQQIRLQAEAFQARLKSWFEPLVEDMQRQWAGLVEKVQAAVGTSAAPVPSDNH

SEQ ID NO: 289 - protein, 308 aa, synthetic construct
FIGITELXKGGGGSGGGSPEPELRQQTEWQSGQRWELALGRFWDYLRWVQTLSEQVQEELLSSQVTQELRALMDETMKELKAYKSELEEQLTPVAEETRARLSKELQAAQARLGADMEDVCGRLVQYRGEVQAMLGQSTEELRVSLASHLRKLRKRLLRDADDLQKCLAVYQAGAREGAERGLSAIRERLGPLVEQGRVRAATVGSLAGQPLQERAQAWGERLRARMEEMGSRTRDRLDEVKEQVAEVRAKLEEQAQQIRLQAEAFQARLKSWFEPLVEDMQRQWAGLVEKVQAAVGTSAAPVPSDNH

SEQ ID NO: 290 - protein, 312 aa, synthetic construct
FIGITELXKGGGGSGGGSGGGSPEPELRQQTEWQSGQRWELALGRFWDYLRWVQTLSEQVQEELLSSQVTQELRALMDETMKELKAYKSELEEQLTPVAEETRARLSKELQAAQARLGADMEDVCGRLVQYRGEVQAMLGQSTEELRVSLASHLRKLRKRLLRDADDLQKCLAVYQAGAREGAERGLSAIRERLGPLVEQGRVRAATVGSLAGQPLQERAQAWGERLRARMEEMGSRTRDRLDEVKEQVAEVRAKLEEQAQQIRLQAEAFQARLKSWFEPLVEDMQRQWAGLVEKVQAAVGTSAAPVPSDNH

SEQ ID NO: 291 - protein, 304 aa, synthetic construct
FIGITELXKEAAAKPEPELRQQTEWQSGQRWELALGRFWDYLRWVQTLSEQVQEELLSSQVTQELRALMDETMKELKAYKSELEEQLTPVAEETRARLSKELQAAQARLGADMEDVCGRLVQYRGEVQAMLGQSTEELRVSLASHLRKLRKRLLRDADDLQKCLAVYQAGAREGAERGLSAIRERLGPLVEQGRVRAATVGSLAGQPLQERAQAWGERLRARMEEMGSRTRDRLDEVKEQVAEVRAKLEEQAQQIRLQAEAFQARLKSWFEPLVEDMQRQWAGLVEKVQAAVGTSAAPVPSDNH

SEQ ID NO: 292 - protein, 309 aa, synthetic construct
FIGITELXKEAAAKEAAAKPEPELRQQTEWQSGQRWELALGRFWDYLRWVQTLSEQVQEELLSSQVTQELRALMDETMKELKAYKSELEEQLTPVAEETRARLSKELQAAQARLGADMEDVCGRLVQYRGEVQAMLGQSTEELRVSLASHLRKLRKRLLRDADDLQKCLAVYQAGAREGAERGLSAIRERLGPLVEQGRVRAATVGSLAGQPLQERAQAWGERLRARMEEMGSRTRDRLDEVKEQVAEVRAKLEEQAQQIRLQAEAFQARLKSWFEPLVEDMQRQWAGLVEKVQAAVGTSAAPVPSDNH

SEQ ID NO: 293 - protein, 314 aa, synthetic construct
FIGITELXKEAAAKEAAAKEAAAKPEPELRQQTEWQSGQRWELALGRFWDYLRWVQTLSEQVQEELLSSQVTQELRALMDETMKELKAYKSELEEQLTPVAEETRARLSKELQAAQARLGADMEDVCGRLVQYRGEVQAMLGQSTEELRVSLASHLRKLRKRLLRDADDLQKCLAVYQAGAREGAERGLSAIRERLGPLVEQGRVRAATVGSLAGQPLQERAQAWGERLRARMEEMGSRTRDRLDEVKEQVAEVRAKLEEQAQQIRLQAEAFQARLKSWFEPLVEDMQRQWAGLVEKVQAAVGTSAAPVPSDNH

SEQ ID NO: 294 - protein, 302 aa, synthetic construct
FIGITELXKGGSPEPELRQQTEWQSGQRWELALGRFWDYLRWVQTLSEQVQEELLSSQVTQELRALMDETMKELKAYKSELEEQLTPVAEETRARLSKELQAAQARLGADMEDVCGRLVQYRGEVQAMLGQSTEELRVSLASHLRKLRKRLLRDADDLQKCLAVYQAGAREGAERGLSAIRERLGPLVEQGRVRAATVGSLAGQPLQERAQAWGERLRARMEEMGSRTRDRLDEVKEQVAEVRAKLEEQAQQIRLQAEAFQARLKSWFEPLVEDMQRQWAGLVEKVQAAVGTSAAPVPSDNH

SEQ ID NO: 295 - protein, 302 aa, synthetic construct
FIGITELXKAAAPEPELRQQTEWQSGQRWELALGRFWDYLRWVQTLSEQVQEELLSSQVTQELRALMDETMKELKAYKSELEEQLTPVAEETRARLSKELQAAQARLGADMEDVCGRLVQYRGEVQAMLGQSTEELRVSLASHLRKLRKRLLRDADDLQKCLAVYQAGAREGAERGLSAIRERLGPLVEQGRVRAATVGSLAGQPLQERAQAWGERLRARMEEMGSRTRDRLDEVKEQVAEVRAKLEEQAQQIRLQAEAFQARLKSWFEPLVEDMQRQWAGLVEKVQAAVGTSAAPVPSDNH

SEQ ID NO: 296 - protein, 303 aa, synthetic construct
FIGITELXKAAAYPEPELRQQTEWQSGQRWELALGRFWDYLRWVQTLSEQVQEELLSSQVTQELRALMDETMKELKAYKSELEEQLTPVAEETRARLSKELQAAQARLGADMEDVCGRLVQYRGEVQAMLGQSTEELRVSLASHLRKLRKRLLRDADDLQKCLAVYQAGAREGAERGLSAIRERLGPLVEQGRVRAATVGSLAGQPLQERAQAWGERLRARMEEMGSRTRDRLDEVKEQVAEVRAKLEEQAQQIRLQAEAFQARLKSWFEPLVEDMQRQWAGLVEKVQAAVGTSAAPVPSDNH

SEQ ID NO: 297 - protein, 299 aa, synthetic construct
FIGITELKKPEPELRQQTEWQSGQRWELALGRFWDYLRWVQTLSEQVQEELLSSQVTQELRALMDETMKELKAYKSELEEQLTPVAEETRARLSKELQAAQARLGADMEDVCGRLVQYRGEVQAMLGQSTEELRVSLASHLRKLRKRLLRDADDLQKCLAVYQAGAREGAERGLSAIRERLGPLVEQGRVRAATVGSLAGQPLQERAQAWGERLRARMEEMGSRTRDRLDEVKEQVAEVRAKLEEQAQQIRLQAEAFQARLKSWFEPLVEDMQRQWAGLVEKVQAAVGTSAAPVPSDNH

SEQ ID NO: 298 - protein, 304 aa, synthetic construct
FIGITELKKGGGGSPEPELRQQTEWQSGQRWELALGRFWDYLRWVQTLSEQVQEELLSSQVTQELRALMDETMKELKAYKSELEEQLTPVAEETRARLSKELQAAQARLGADMEDVCGRLVQYRGEVQAMLGQSTEELRVSLASHLRKLRKRLLRDADDLQKCLAVYQAGAREGAERGLSAIRERLGPLVEQGRVRAATVGSLAGQPLQERAQAWGERLRARMEEMGSRTRDRLDEVKEQVAEVRAKLEEQAQQIRLQAEAFQARLKSWFEPLVEDMQRQWAGLVEKVQAAVGTSAAPVPSDNH

SEQ ID NO: 299 - protein, 308 aa, synthetic construct
FIGITELKKGGGGSGGGSPEPELRQQTEWQSGQRWELALGRFWDYLRWVQTLSEQVQEELLSSQVTQELRALMDETMKELKAYKSELEEQLTPVAEETRARLSKELQAAQARLGADMEDVCGRLVQYRGEVQAMLGQSTEELRVSLASHLRKLRKRLLRDADDLQKCLAVYQAGAREGAERGLSAIRERLGPLVEQGRVRAATVGSLAGQPLQERAQAWGERLRARMEEMGSRTRDRLDEVKEQVAEVRAKLEEQAQQIRLQAEAFQARLKSWFEPLVEDMQRQWAGLVEKVQAAVGTSAAPVPSDNH

SEQ ID NO: 300 - protein, 312 aa, synthetic construct
FIGITELKKGGGGSGGGSGGGSPEPELRQQTEWQSGQRWELALGRFWDYLRWVQTLSEQVQEELLSSQVTQELRALMDETMKELKAYKSELEEQLTPVAEETRARLSKELQAAQARLGADMEDVCGRLVQYRGEVQAMLGQSTEELRVSLASHLRKLRKRLLRDADDLQKCLAVYQAGAREGAERGLSAIRERLGPLVEQGRVRAATVGSLAGQPLQERAQAWGERLRARMEEMGSRTRDRLDEVKEQVAEVRAKLEEQAQQIRLQAEAFQARLKSWFEPLVEDMQRQWAGLVEKVQAAVGTSAAPVPSDNH

SEQ ID NO: 301 - protein, 304 aa, synthetic construct
FIGITELKKEAAAKPEPELRQQTEWQSGQRWELALGRFWDYLRWVQTLSEQVQEELLSSQVTQELRALMDETMKELKAYKSELEEQLTPVAEETRARLSKELQAAQARLGADMEDVCGRLVQYRGEVQAMLGQSTEELRVSLASHLRKLRKRLLRDADDLQKCLAVYQAGAREGAERGLSAIRERLGPLVEQGRVRAATVGSLAGQPLQERAQAWGERLRARMEEMGSRTRDRLDEVKEQVAEVRAKLEEQAQQIRLQAEAFQARLKSWFEPLVEDMQRQWAGLVEKVQAAVGTSAAPVPSDNH

SEQ ID NO: 302 - protein, 309 aa, synthetic construct
FIGITELKKEAAAKEAAAKPEPELRQQTEWQSGQRWELALGRFWDYLRWVQTLSEQVQEELLSSQVTQELRALMDETMKELKAYKSELEEQLTPVAEETRARLSKELQAAQARLGADMEDVCGRLVQYRGEVQAMLGQSTEELRVSLASHLRKLRKRLLRDADDLQKCLAVYQAGAREGAERGLSAIRERLGPLVEQGRVRAATVGSLAGQPLQERAQAWGERLRARMEEMGSRTRDRLDEVKEQVAEVRAKLEEQAQQIRLQAEAFQARLKSWFEPLVEDMQRQWAGLVEKVQAAVGTSAAPVPSDNH

SEQ ID NO: 303 - protein, 314 aa, synthetic construct
FIGITELKKEAAAKEAAAKEAAAKPEPELRQQTEWQSGQRWELALGRFWDYLRWVQTLSEQVQEELLSSQVTQELRALMDETMKELKAYKSELEEQLTPVAEETRARLSKELQAAQARLGADMEDVCGRLVQYRGEVQAMLGQSTEELRVSLASHLRKLRKRLLRDADDLQKCLAVYQAGAREGAERGLSAIRERLGPLVEQGRVRAATVGSLAGQPLQERAQAWGERLRARMEEMGSRTRDRLDEVKEQVAEVRAKLEEQAQQIRLQAEAFQARLKSWFEPLVEDMQRQWAGLVEKVQAAVGTSAAPVPSDNH

SEQ ID NO: 304 - protein, 302 aa, synthetic construct
FIGITELKKGGSPEPELRQQTEWQSGQRWELALGRFWDYLRWVQTLSEQVQEELLSSQVTQELRALMDETMKELKAYKSELEEQLTPVAEETRARLSKELQAAQARLGADMEDVCGRLVQYRGEVQAMLGQSTEELRVSLASHLRKLRKRLLRDADDLQKCLAVYQAGAREGAERGLSAIRERLGPLVEQGRVRAATVGSLAGQPLQERAQAWGERLRARMEEMGSRTRDRLDEVKEQVAEVRAKLEEQAQQIRLQAEAFQARLKSWFEPLVEDMQRQWAGLVEKVQAAVGTSAAPVPSDNH

SEQ ID NO: 305 - protein, 302 aa, synthetic construct
FIGITELKKAAAPEPELRQQTEWQSGQRWELALGRFWDYLRWVQTLSEQVQEELLSSQVTQELRALMDETMKELKAYKSELEEQLTPVAEETRARLSKELQAAQARLGADMEDVCGRLVQYRGEVQAMLGQSTEELRVSLASHLRKLRKRLLRDADDLQKCLAVYQAGAREGAERGLSAIRERLGPLVEQGRVRAATVGSLAGQPLQERAQAWGERLRARMEEMGSRTRDRLDEVKEQVAEVRAKLEEQAQQIRLQAEAFQARLKSWFEPLVEDMQRQWAGLVEKVQAAVGTSAAPVPSDNH

SEQ ID NO: 306 - protein, 303 aa, synthetic construct
FIGITELKKAAAYPEPELRQQTEWQSGQRWELALGRFWDYLRWVQTLSEQVQEELLSSQVTQELRALMDETMKELKAYKSELEEQLTPVAEETRARLSKELQAAQARLGADMEDVCGRLVQYRGEVQAMLGQSTEELRVSLASHLRKLRKRLLRDADDLQKCLAVYQAGAREGAERGLSAIRERLGPLVEQGRVRAATVGSLAGQPLQERAQAWGERLRARMEEMGSRTRDRLDEVKEQVAEVRAKLEEQAQQIRLQAEAFQARLKSWFEPLVEDMQRQWAGLVEKVQAAVGTSAAPVPSDNH

SEQ ID NO: 307 - protein, 299 aa, synthetic construct
FIGITELLKPEPELRQQTEWQSGQRWELALGRFWDYLRWVQTLSEQVQEELLSSQVTQELRALMDETMKELKAYKSELEEQLTPVAEETRARLSKELQAAQARLGADMEDVCGRLVQYRGEVQAMLGQSTEELRVSLASHLRKLRKRLLRDADDLQKCLAVYQAGAREGAERGLSAIRERLGPLVEQGRVRAATVGSLAGQPLQERAQAWGERLRARMEEMGSRTRDRLDEVKEQVAEVRAKLEEQAQQIRLQAEAFQARLKSWFEPLVEDMQRQWAGLVEKVQAAVGTSAAPVPSDNH

SEQ ID NO: 308 - protein, 304 aa, synthetic construct
FIGITELLKGGGGSPEPELRQQTEWQSGQRWELALGRFWDYLRWVQTLSEQVQEELLSSQVTQELRALMDETMKELKAYKSELEEQLTPVAEETRARLSKELQAAQARLGADMEDVCGRLVQYRGEVQAMLGQSTEELRVSLASHLRKLRKRLLRDADDLQKCLAVYQAGAREGAERGLSAIRERLGPLVEQGRVRAATVGSLAGQPLQERAQAWGERLRARMEEMGSRTRDRLDEVKEQVAEVRAKLEEQAQQIRLQAEAFQARLKSWFEPLVEDMQRQWAGLVEKVQAAVGTSAAPVPSDNH

SEQ ID NO: 309 - protein, 308 aa, synthetic construct
FIGITELLKGGGGSGGGSPEPELRQQTEWQSGQRWELALGRFWDYLRWVQTLSEQVQEELLSSQVTQELRALMDETMKELKAYKSELEEQLTPVAEETRARLSKELQAAQARLGADMEDVCGRLVQYRGEVQAMLGQSTEELRVSLASHLRKLRKRLLRDADDLQKCLAVYQAGAREGAERGLSAIRERLGPLVEQGRVRAATVGSLAGQPLQERAQAWGERLRARMEEMGSRTRDRLDEVKEQVAEVRAKLEEQAQQIRLQAEAFQARLKSWFEPLVEDMQRQWAGLVEKVQAAVGTSAAPVPSDNH

SEQ ID NO: 310 - protein, 312 aa, synthetic construct
FIGITELLKGGGGSGGGSGGGSPEPELRQQTEWQSGQRWELALGRFWDYLRWVQTLSEQVQEELLSSQVTQELRALMDETMKELKAYKSELEEQLTPVAEETRARLSKELQAAQARLGADMEDVCGRLVQYRGEVQAMLGQSTEELRVSLASHLRKLRKRLLRDADDLQKCLAVYQAGAREGAERGLSAIRERLGPLVEQGRVRAATVGSLAGQPLQERAQAWGERLRARMEEMGSRTRDRLDEVKEQVAEVRAKLEEQAQQIRLQAEAFQARLKSWFEPLVEDMQRQWAGLVEKVQAAVGTSAAPVPSDNH

SEQ ID NO: 311 - protein, 304 aa, synthetic construct
FIGITELLKEAAAKPEPELRQQTEWQSGQRWELALGRFWDYLRWVQTLSEQVQEELLSSQVTQELRALMDETMKELKAYKSELEEQLTPVAEETRARLSKELQAAQARLGADMEDVCGRLVQYRGEVQAMLGQSTEELRVSLASHLRKLRKRLLRDADDLQKCLAVYQAGAREGAERGLSAIRERLGPLVEQGRVRAATVGSLAGQPLQERAQAWGERLRARMEEMGSRTRDRLDEVKEQVAEVRAKLEEQAQQIRLQAEAFQARLKSWFEPLVEDMQRQWAGLVEKVQAAVGTSAAPVPSDNH

SEQ ID NO: 312 - protein, 309 aa, synthetic construct
FIGITELLKEAAAKEAAAKPEPELRQQTEWQSGQRWELALGRFWDYLRWVQTLSEQVQEELLSSQVTQELRALMDETMKELKAYKSELEEQLTPVAEETRARLSKELQAAQARLGADMEDVCGRLVQYRGEVQAMLGQSTEELRVSLASHLRKLRKRLLRDADDLQKCLAVYQAGAREGAERGLSAIRERLGPLVEQGRVRAATVGSLAGQPLQERAQAWGERLRARMEEMGSRTRDRLDEVKEQVAEVRAKLEEQAQQIRLQAEAFQARLKSWFEPLVEDMQRQWAGLVEKVQAAVGTSAAPVPSDNH

SEQ ID NO: 313 - protein, 314 aa, synthetic construct
FIGITELLKEAAAKEAAAKEAAAKPEPELRQQTEWQSGQRWELALGRFWDYLRWVQTLSEQVQEELLSSQVTQELRALMDETMKELKAYKSELEEQLTPVAEETRARLSKELQAAQARLGADMEDVCGRLVQYRGEVQAMLGQSTEELRVSLASHLRKLRKRLLRDADDLQKCLAVYQAGAREGAERGLSAIRERLGPLVEQGRVRAATVGSLAGQPLQERAQAWGERLRARMEEMGSRTRDRLDEVKEQVAEVRAKLEEQAQQIRLQAEAFQARLKSWFEPLVEDMQRQWAGLVEKVQAAVGTSAAPVPSDNH

SEQ ID NO: 314 - protein, 302 aa, synthetic construct
FIGITELLKGGSPEPELRQQTEWQSGQRWELALGRFWDYLRWVQTLSEQVQEELLSSQVTQELRALMDETMKELKAYKSELEEQLTPVAEETRARLSKELQAAQARLGADMEDVCGRLVQYRGEVQAMLGQSTEELRVSLASHLRKLRKRLLRDADDLQKCLAVYQAGAREGAERGLSAIRERLGPLVEQGRVRAATVGSLAGQPLQERAQAWGERLRARMEEMGSRTRDRLDEVKEQVAEVRAKLEEQAQQIRLQAEAFQARLKSWFEPLVEDMQRQWAGLVEKVQAAVGTSAAPVPSDNH

SEQ ID NO: 315 - protein, 302 aa, synthetic construct
FIGITELLKAAAPEPELRQQTEWQSGQRWELALGRFWDYLRWVQTLSEQVQEELLSSQVTQELRALMDETMKELKAYKSELEEQLTPVAEETRARLSKELQAAQARLGADMEDVCGRLVQYRGEVQAMLGQSTEELRVSLASHLRKLRKRLLRDADDLQKCLAVYQAGAREGAERGLSAIRERLGPLVEQGRVRAATVGSLAGQPLQERAQAWGERLRARMEEMGSRTRDRLDEVKEQVAEVRAKLEEQAQQIRLQAEAFQARLKSWFEPLVEDMQRQWAGLVEKVQAAVGTSAAPVPSDNH

SEQ ID NO: 316 - protein, 303 aa, synthetic construct
FIGITELLKAAAYPEPELRQQTEWQSGQRWELALGRFWDYLRWVQTLSEQVQEELLSSQVTQELRALMDETMKELKAYKSELEEQLTPVAEETRARLSKELQAAQARLGADMEDVCGRLVQYRGEVQAMLGQSTEELRVSLASHLRKLRKRLLRDADDLQKCLAVYQAGAREGAERGLSAIRERLGPLVEQGRVRAATVGSLAGQPLQERAQAWGERLRARMEEMGSRTRDRLDEVKEQVAEVRAKLEEQAQQIRLQAEAFQARLKSWFEPLVEDMQRQWAGLVEKVQAAVGTSAAPVPSDNH

SEQ ID NO: 317 - protein, 299 aa, synthetic construct
FIGITELHKPEPELRQQTEWQSGQRWELALGRFWDYLRWVQTLSEQVQEELLSSQVTQELRALMDETMKELKAYKSELEEQLTPVAEETRARLSKELQAAQARLGADMEDVCGRLVQYRGEVQAMLGQSTEELRVSLASHLRKLRKRLLRDADDLQKCLAVYQAGAREGAERGLSAIRERLGPLVEQGRVRAATVGSLAGQPLQERAQAWGERLRARMEEMGSRTRDRLDEVKEQVAEVRAKLEEQAQQIRLQAEAFQARLKSWFEPLVEDMQRQWAGLVEKVQAAVGTSAAPVPSDNH

SEQ ID NO: 318 - protein, 304 aa, synthetic construct
FIGITELHKGGGGSPEPELRQQTEWQSGQRWELALGRFWDYLRWVQTLSEQVQEELLSSQVTQELRALMDETMKELKAYKSELEEQLTPVAEETRARLSKELQAAQARLGADMEDVCGRLVQYRGEVQAMLGQSTEELRVSLASHLRKLRKRLLRDADDLQKCLAVYQAGAREGAERGLSAIRERLGPLVEQGRVRAATVGSLAGQPLQERAQAWGERLRARMEEMGSRTRDRLDEVKEQVAEVRAKLEEQAQQIRLQAEAFQARLKSWFEPLVEDMQRQWAGLVEKVQAAVGTSAAPVPSDNH

SEQ ID NO: 319 - protein, 308 aa, synthetic construct
FIGITELHKGGGGSGGGSPEPELRQQTEWQSGQRWELALGRFWDYLRWVQTLSEQVQEELLSSQVTQELRALMDETMKELKAYKSELEEQLTPVAEETRARLSKELQAAQARLGADMEDVCGRLVQYRGEVQAMLGQSTEELRVSLASHLRKLRKRLLRDADDLQKCLAVYQAGAREGAERGLSAIRERLGPLVEQGRVRAATVGSLAGQPLQERAQAWGERLRARMEEMGSRTRDRLDEVKEQVAEVRAKLEEQAQQIRLQAEAFQARLKSWFEPLVEDMQRQWAGLVEKVQAAVGTSAAPVPSDNH

SEQ ID NO: 320 - protein, 312 aa, synthetic construct
FIGITELHKGGGGSGGGSGGGSPEPELRQQTEWQSGQRWELALGRFWDYLRWVQTLSEQVQEELLSSQVTQELRALMDETMKELKAYKSELEEQLTPVAEETRARLSKELQAAQARLGADMEDVCGRLVQYRGEVQAMLGQSTEELRVSLASHLRKLRKRLLRDADDLQKCLAVYQAGAREGAERGLSAIRERLGPLVEQGRVRAATVGSLAGQPLQERAQAWGERLRARMEEMGSRTRDRLDEVKEQVAEVRAKLEEQAQQIRLQAEAFQARLKSWFEPLVEDMQRQWAGLVEKVQAAVGTSAAPVPSDNH

SEQ ID NO: 321 - protein, 304 aa, synthetic construct
FIGITELHKEAAAKPEPELRQQTEWQSGQRWELALGRFWDYLRWVQTLSEQVQEELLSSQVTQELRALMDETMKELKAYKSELEEQLTPVAEETRARLSKELQAAQARLGADMEDVCGRLVQYRGEVQAMLGQSTEELRVSLASHLRKLRKRLLRDADDLQKCLAVYQAGAREGAERGLSAIRERLGPLVEQGRVRAATVGSLAGQPLQERAQAWGERLRARMEEMGSRTRDRLDEVKEQVAEVRAKLEEQAQQIRLQAEAFQARLKSWFEPLVEDMQRQWAGLVEKVQAAVGTSAAPVPSDNH

SEQ ID NO: 322 - protein, 309 aa, synthetic construct
FIGITELHKEAAAKEAAAKPEPELRQQTEWQSGQRWELALGRFWDYLRWVQTLSEQVQEELLSSQVTQELRALMDETMKELKAYKSELEEQLTPVAEETRARLSKELQAAQARLGADMEDVCGRLVQYRGEVQAMLGQSTEELRVSLASHLRKLRKRLLRDADDLQKCLAVYQAGAREGAERGLSAIRERLGPLVEQGRVRAATVGSLAGQPLQERAQAWGERLRARMEEMGSRTRDRLDEVKEQVAEVRAKLEEQAQQIRLQAEAFQARLKSWFEPLVEDMQRQWAGLVEKVQAAVGTSAAPVPSDNH

SEQ ID NO: 323 - protein, 314 aa, synthetic construct
FIGITELHKEAAAKEAAAKEAAAKPEPELRQQTEWQSGQRWELALGRFWDYLRWVQTLSEQVQEELLSSQVTQELRALMDETMKELKAYKSELEEQLTPVAEETRARLSKELQAAQARLGADMEDVCGRLVQYRGEVQAMLGQSTEELRVSLASHLRKLRKRLLRDADDLQKCLAVYQAGAREGAERGLSAIRERLGPLVEQGRVRAATVGSLAGQPLQERAQAWGERLRARMEEMGSRTRDRLDEVKEQVAEVRAKLEEQAQQIRLQAEAFQARLKSWFEPLVEDMQRQWAGLVEKVQAAVGTSAAPVPSDNH

SEQ ID NO: 324 - protein, 302 aa, synthetic construct
FIGITELHKAAAPEPELRQQTEWQSGQRWELALGRFWDYLRWVQTLSEQVQEELLSSQVTQELRALMDETMKELKAYKSELEEQLTPVAEETRARLSKELQAAQARLGADMEDVCGRLVQYRGEVQAMLGQSTEELRVSLASHLRKLRKRLLRDADDLQKCLAVYQAGAREGAERGLSAIRERLGPLVEQGRVRAATVGSLAGQPLQERAQAWGERLRARMEEMGSRTRDRLDEVKEQVAEVRAKLEEQAQQIRLQAEAFQARLKSWFEPLVEDMQRQWAGLVEKVQAAVGTSAAPVPSDNH

SEQ ID NO: 325 - protein, 302 aa, synthetic construct; identical to SEQ ID NO: 315

SEQ ID NO: 326 - protein, 302 aa, synthetic construct; identical to SEQ ID NO: 324

SEQ ID NO: 327 - skipped

SEQ ID NO: 328 - protein, 4 aa, synthetic construct
GFLG

SEQ ID NO: 329 - protein, 6 aa, synthetic construct
PLGLWA

SEQ ID NO: 330 - protein, 10 aa, synthetic construct
AGNRVRRSVG

SEQ ID NO: 331 - protein, 312 aa, synthetic construct
FIGITELKKGFLGKVEQAVETEPEPELRQQTEWQSGQRWELALGRFWDYLRWVQTLSEQVQEELLSSQVTQELRALMDETMKELKAYKSELEEQLTPVAEETRARLSKELQAAQARLGADMEDVCGRLVQYRGEVQAMLGQSTEELRVSLASHLRKLRKRLLRDADDLQKCLAVYQAGAREGAERGLSAIRERLGPLVEQGRVRAATVGSLAGQPLQERAQAWGERLRARMEEMGSRTRDRLDEVKEQVAEVRAKLEEQAQQIRLQAEAFQARLKSWFEPLVEDMQRQWAGLVEKVQAAVGTSAAPVPSDNH

SEQ ID NO: 332 - protein, 314 aa, synthetic construct
FIGITELKKPLGLWAKVEQAVETEPEPELRQQTEWQSGQRWELALGRFWDYLRWVQTLSEQVQEELLSSQVTQELRALMDETMKELKAYKSELEEQLTPVAEETRARLSKELQAAQARLGADMEDVCGRLVQYRGEVQAMLGQSTEELRVSLASHLRKLRKRLLRDADDLQKCLAVYQAGAREGAERGLSAIRERLGPLVEQGRVRAATVGSLAGQPLQERAQAWGERLRARMEEMGSRTRDRLDEVKEQVAEVRAKLEEQAQQIRLQAEAFQARLKSWFEPLVEDMQRQWAGLVEKVQAAVGTSAAPVPSDNH

SEQ ID NO: 333 - protein, 318 aa, synthetic construct
FIGITELKKAGNRVRRSVGKVEQAVETEPEPELRQQTEWQSGQRWELALGRFWDYLRWVQTLSEQVQEELLSSQVTQELRALMDETMKELKAYKSELEEQLTPVAEETRARLSKELQAAQARLGADMEDVCGRLVQYRGEVQAMLGQSTEELRVSLASHLRKLRKRLLRDADDLQKCLAVYQAGAREGAERGLSAIRERLGPLVEQGRVRAATVGSLAGQPLQERAQAWGERLRARMEEMGSRTRDRLDEVKEQVAEVRAKLEEQAQQIRLQAEAFQARLKSWFEPLVEDMQRQWAGLVEKVQAAVGTSAAPVPSDNH

SEQ ID NO: 334 - protein, 122 aa, synthetic construct
FIGITELKKGFLGRAATVGSLAGQPLQERAQAWGERLRARMEEMGSRTRDRLDEVKEQVAEVRAKLEEQAQQIRLQAEAFQARLKSWFEPLVEDMQRQWAGLVEKVQAAVGTSAAPVPSDNH

SEQ ID NO: 335 - protein, 124 aa, synthetic construct
FIGITELKKPLGLWARAATVGSLAGQPLQERAQAWGERLRARMEEMGSRTRDRLDEVKEQVAEVRAKLEEQAQQIRLQAEAFQARLKSWFEPLVEDMQRQWAGLVEKVQAAVGTSAAPVPSDNH

SEQ ID NO: 336 - protein, 128 aa, synthetic construct
FIGITELKKAGNRVRRSVGRAATVGSLAGQPLQERAQAWGERLRARMEEMGSRTRDRLDEVKEQVAEVRAKLEEQAQQIRLQAEAFQARLKSWFEPLVEDMQRQWAGLVEKVQAAVGTSAAPVPSDNH

SEQ ID NO: 337 - protein, 149 aa, synthetic construct
FIGITELKKGFLGAGAREGAERGLSAIRERLGPLVEQGRVRAATVGSLAGQPLQERAQAWGERLRARMEEMGSRTRDRLDEVKEQVAEVRAKLEEQAQQIRLQAEAFQARLKSWFEPLVEDMQRQWAGLVEKVQAAVGTSAAPVPSDNH

SEQ ID NO: 338 - protein, 151 aa, synthetic construct
FIGITELKKPLGLWAAGAREGAERGLSAIRERLGPLVEQGRVRAATVGSLAGQPLQERAQAWGERLRARMEEMGSRTRDRLDEVKEQVAEVRAKLEEQAQQIRLQAEAFQARLKSWFEPLVEDMQRQWAGLVEKVQAAVGTSAAPVPSDNH

SEQ ID NO: 339 - protein, 155 aa, synthetic construct
FIGITELKKAGNRVRRSVGAGAREGAERGLSAIRERLGPLVEQGRVRAATVGSLAGQPLQERAQAWGERLRARMEEMGSRTRDRLDEVKEQVAEVRAKLEEQAQQIRLQAEAFQARLKSWFEPLVEDMQRQWAGLVEKVQAAVGTSAAPVPSDNH

SEQ ID NO: 340 - protein, 269 aa, synthetic construct
FIGITELKKGFLGSEQVQEELLSSQVTQELRALMDETMKELKAYKSELEEQLTPVAEETRARLSKELQAAQARLGADMEDVCGRLVQYRGEVQAMLGQSTEELRVSLASHLRKLRKRLLRDADDLQKCLAVYQAGAREGAERGLSAIRERLGPLVEQGRVRAATVGSLAGQPLQERAQAWGERLRARMEEMGSRTRDRLDEVKEQVAEVRAKLEEQAQQIRLQAEAFQARLKSWFEPLVEDMQRQWAGLVEKVQAAVGTSAAPVPSDNH

SEQ ID NO: 341 - protein, 271 aa, synthetic construct
FIGITELKKPLGLWASEQVQEELLSSQVTQELRALMDETMKELKAYKSELEEQLTPVAEETRARLSKELQAAQARLGADMEDVCGRLVQYRGEVQAMLGQSTEELRVSLASHLRKLRKRLLRDADDLQKCLAVYQAGAREGAERGLSAIRERLGPLVEQGRVRAATVGSLAGQPLQERAQAWGERLRARMEEMGSRTRDRLDEVKEQVAEVRAKLEEQAQQIRLQAEAFQARLKSWFEPLVEDMQRQWAGLVEKVQAAVGTSAAPVPSDNH

SEQ ID NO: 342 - protein, 275 aa, synthetic construct
FIGITELKKAGNRVRRSVGSEQVQEELLSSQVTQELRALMDETMKELKAYKSELEEQLTPVAEETRARLSKELQAAQARLGADMEDVCGRLVQYRGEVQAMLGQSTEELRVSLASHLRKLRKRLLRDADDLQKCLAVYQAGAREGAERGLSAIRERLGPLVEQGRVRAATVGSLAGQPLQERAQAWGERLRARMEEMGSRTRDRLDEVKEQVAEVRAKLEEQAQQIRLQAEAFQARLKSWFEPLVEDMQRQWAGLVEKVQAAVGTSAAPVPSDNH

SEQ ID NO: 343 - protein, 259 aa, synthetic construct
FIGITELKKGFLGSQVTQELRALMDETMKELKAYKSELEEQLTPVAEETRARLSKELQAAQARLGADMEDVCGRLVQYRGEVQAMLGQSTEELRVSLASHLRKLRKRLLRDADDLQKCLAVYQAGAREGAERGLSAIRERLGPLVEQGRVRAATVGSLAGQPLQERAQAWGERLRARMEEMGSRTRDRLDEVKEQVAEVRAKLEEQAQQIRLQAEAFQARLKSWFEPLVEDMQRQWAGLVEKVQAAVGTSAAPVPSDNH

SEQ ID NO: 344 - protein, 261 aa, synthetic construct
FIGITELKKPLGLWASQVTQELRALMDETMKELKAYKSELEEQLTPVAEETRARLSKELQAAQARLGADMEDVCGRLVQYRGEVQAMLGQSTEELRVSLASHLRKLRKRLLRDADDLQKCLAVYQAGAREGAERGLSAIRERLGPLVEQGRVRAATVGSLAGQPLQERAQAWGERLRARMEEMGSRTRDRLDEVKEQVAEVRAKLEEQAQQIRLQAEAFQARLKSWFEPLVEDMQRQWAGLVEKVQAAVGTSAAPVPSDNH

SEQ ID NO: 345 - protein, 265 aa, synthetic construct
FIGITELKKAGNRVRRSVGSQVTQELRALMDETMKELKAYKSELEEQLTPVAEETRARLSKELQAAQARLGADMEDVCGRLVQYRGEVQAMLGQSTEELRVSLASHLRKLRKRLLRDADDLQKCLAVYQAGAREGAERGLSAIRERLGPLVEQGRVRAATVGSLAGQPLQERAQAWGERLRARMEEMGSRTRDRLDEVKEQVAEVRAKLEEQAQQIRLQAEAFQARLKSWFEPLVEDMQRQWAGLVEKVQAAVGTSAAPVPSDNH

SEQ ID NO: 346 - protein, 303 aa, synthetic construct
FIGITELKKGFLGPEPELRQQTEWQSGQRWELALGRFWDYLRWVQTLSEQVQEELLSSQVTQELRALMDETMKELKAYKSELEEQLTPVAEETRARLSKELQAAQARLGADMEDVCGRLVQYRGEVQAMLGQSTEELRVSLASHLRKLRKRLLRDADDLQKCLAVYQAGAREGAERGLSAIRERLGPLVEQGRVRAATVGSLAGQPLQERAQAWGERLRARMEEMGSRTRDRLDEVKEQVAEVRAKLEEQAQQIRLQAEAFQARLKSWFEPLVEDMQRQWAGLVEKVQAAVGTSAAPVPSDNH

SEQ ID NO: 347 - protein, 305 aa, synthetic construct
FIGITELKKPLGLWAPEPELRQQTEWQSGQRWELALGRFWDYLRWVQTLSEQVQEELLSSQVTQELRALMDETMKELKAYKSELEEQLTPVAEETRARLSKELQAAQARLGADMEDVCGRLVQYRGEVQAMLGQSTEELRVSLASHLRKLRKRLLRDADDLQKCLAVYQAGAREGAERGLSAIRERLGPLVEQGRVRAATVGSLAGQPLQERAQAWGERLRARMEEMGSRTRDRLDEVKEQVAEVRAKLEEQAQQIRLQAEAFQARLKSWFEPLVEDMQRQWAGLVEKVQAAVGTSAAPVPSDNH

SEQ ID NO: 348 - protein, 309 aa, synthetic construct
FIGITELKKAGNRVRRSVGPEPELRQQTEWQSGQRWELALGRFWDYLRWVQTLSEQVQEELLSSQVTQELRALMDETMKELKAYKSELEEQLTPVAEETRARLSKELQAAQARLGADMEDVCGRLVQYRGEVQAMLGQSTEELRVSLASHLRKLRKRLLRDADDLQKCLAVYQAGAREGAERGLSAIRERLGPLVEQGRVRAATVGSLAGQPLQERAQAWGERLRARMEEMGSRTRDRLDEVKEQVAEVRAKLEEQAQQIRLQAEAFQARLKSWFEPLVEDMQRQWAGLVEKVQAAVGTSAAPVPSDNH

SEQ ID NO: 349 - protein, 312 aa, synthetic construct
FIGITELLKGFLGKVEQAVETEPEPELRQQTEWQSGQRWELALGRFWDYLRWVQTLSEQVQEELLSSQVTQELRALMDETMKELKAYKSELEEQLTPVAEETRARLSKELQAAQARLGADMEDVCGRLVQYRGEVQAMLGQSTEELRVSLASHLRKLRKRLLRDADDLQKCLAVYQAGAREGAERGLSAIRERLGPLVEQGRVRAATVGSLAGQPLQERAQAWGERLRARMEEMGSRTRDRLDEVKEQVAEVRAKLEEQAQQIRLQAEAFQARLKSWFEPLVEDMQRQWAGLVEKVQAAVGTSAAPVPSDNH

SEQ ID NO: 350 - protein, 314 aa, synthetic construct
FIGITELLKPLGLWAKVEQAVETEPEPELRQQTEWQSGQRWELALGRFWDYLRWVQTLSEQVQEELLSSQVTQELRALMDETMKELKAYKSELEEQLTPVAEETRARLSKELQAAQARLGADMEDVCGRLVQYRGEVQAMLGQSTEELRVSLASHLRKLRKRLLRDADDLQKCLAVYQAGAREGAERGLSAIRERLGPLVEQGRVRAATVGSLAGQPLQERAQAWGERLRARMEEMGSRTRDRLDEVKEQVAEVRAKLEEQAQQIRLQAEAFQARLKSWFEPLVEDMQRQWAGLVEKVQAAVGTSAAPVPSDNH

SEQ ID NO: 351 - protein, 318 aa, synthetic construct
FIGITELLKAGNRVRRSVGKVEQAVETEPEPELRQQTEWQSGQRWELALGRFWDYLRWVQTLSEQVQEELLSSQVTQELRALMDETMKELKAYKSELEEQLTPVAEETRARLSKELQAAQARLGADMEDVCGRLVQYRGEVQAMLGQSTEELRVSLASHLRKLRKRLLRDADDLQKCLAVYQAGAREGAERGLSAIRERLGPLVEQGRVRAATVGSLAGQPLQERAQAWGERLRARMEEMGSRTRDRLDEVKEQVAEVRAKLEEQAQQIRLQAEAFQARLKSWFEPLVEDMQRQWAGLVEKVQAAVGTSAAPVPSDNH

SEQ ID NO: 352 - protein, 122 aa, synthetic construct
FIGITELLKGFLGRAATVGSLAGQPLQERAQAWGERLRARMEEMGSRTRDRLDEVKEQVAEVRAKLEEQAQQIRLQAEAFQARLKSWFEPLVEDMQRQWAGLVEKVQAAVGTSAAPVPSDNH

SEQ ID NO: 353 - protein, 124 aa, synthetic construct
FIGITELLKPLGLWARAATVGSLAGQPLQERAQAWGERLRARMEEMGSRTRDRLDEVKEQVAEVRAKLEEQAQQIRLQAEAFQARLKSWFEPLVEDMQRQWAGLVEKVQAAVGTSAAPVPSDNH

SEQ ID NO: 354 - protein, 128 aa, synthetic construct
FIGITELLKAGNRVRRSVGRAATVGSLAGQPLQERAQAWGERLRARMEEMGSRTRDRLDEVKEQVAEVRAKLEEQAQQIRLQAEAFQARLKSWFEPLVEDMQRQWAGLVEKVQAAVGTSAAPVPSDNH

SEQ ID NO: 355 - protein, 149 aa, synthetic construct
FIGITELLKGFLGAGAREGAERGLSAIRERLGPLVEQGRVRAATVGSLAGQPLQERAQAWGERLRARMEEMGSRTRDRLDEVKEQVAEVRAKLEEQAQQIRLQAEAFQARLKSWFEPLVEDMQRQWAGLVEKVQAAVGTSAAPVPSDNH

SEQ ID NO: 356 - protein, 151 aa, synthetic construct
FIGITELLKPLGLWAAGAREGAERGLSAIRERLGPLVEQGRVRAATVGSLAGQPLQERAQAWGERLRARMEEMGSRTRDRLDEVKEQVAEVRAKLEEQAQQIRLQAEAFQARLKSWFEPLVEDMQRQWAGLVEKVQAAVGTSAAPVPSDNH

SEQ ID NO: 357 - protein, 155 aa, synthetic construct
FIGITELLKAGNRVRRSVGAGAREGAERGLSAIRERLGPLVEQGRVRAATVGSLAGQPLQERAQAWGERLRARMEEMGSRTRDRLDEVKEQVAEVRAKLEEQAQQIRLQAEAFQARLKSWFEPLVEDMQRQWAGLVEKVQAAVGTSAAPVPSDNH

SEQ ID NO: 358 - protein, 269 aa, synthetic construct
FIGITELLKGFLGSEQVQEELLSSQVTQELRALMDETMKELKAYKSELEEQLTPVAEETRARLSKELQAAQARLGADMEDVCGRLVQYRGEVQAMLGQSTEELRVSLASHLRKLRKRLLRDADDLQKCLAVYQAGAREGAERGLSAIRERLGPLVEQGRVRAATVGSLAGQPLQERAQAWGERLRARMEEMGSRTRDRLDEVKEQVAEVRAKLEEQAQQIRLQAEAFQARLKSWFEPLVEDMQRQWAGLVEKVQAAVGTSAAPVPSDNH

SEQ ID NO: 359 - protein, 271 aa, synthetic construct
FIGITELLKPLGLWASEQVQEELLSSQVTQELRALMDETMKELKAYKSELEEQLTPVAEETRARLSKELQAAQARLGADMEDVCGRLVQYRGEVQAMLGQSTEELRVSLASHLRKLRKRLLRDADDLQKCLAVYQAGAREGAERGLSAIRERLGPLVEQGRVRAATVGSLAGQPLQERAQAWGERLRARMEEMGSRTRDRLDEVKEQVAEVRAKLEEQAQQIRLQAEAFQARLKSWFEPLVEDMQRQWAGLVEKVQAAVGTSAAPVPSDNH

SEQ ID NO: 360 - protein, 275 aa, synthetic construct
FIGITELLKAGNRVRRSVGSEQVQEELLSSQVTQELRALMDETMKELKAYKSELEEQLTPVAEETRARLSKELQAAQARLGADMEDVCGRLVQYRGEVQAMLGQSTEELRVSLASHLRKLRKRLLRDADDLQKCLAVYQAGAREGAERGLSAIRERLGPLVEQGRVRAATVGSLAGQPLQERAQAWGERLRARMEEMGSRTRDRLDEVKEQVAEVRAKLEEQAQQIRLQAEAFQARLKSWFEPLVEDMQRQWAGLVEKVQAAVGTSAAPVPSDNH

SEQ ID NO: 361 - protein, 259 aa, synthetic construct
FIGITELLKGFLGSQVTQELRALMDETMKELKAYKSELEEQLTPVAEETRARLSKELQAAQARLGADMEDVCGRLVQYRGEVQAMLGQSTEELRVSLASHLRKLRKRLLRDADDLQKCLAVYQAGAREGAERGLSAIRERLGPLVEQGRVRAATVGSLAGQPLQERAQAWGERLRARMEEMGSRTRDRLDEVKEQVAEVRAKLEEQAQQIRLQAEAFQARLKSWFEPLVEDMQRQWAGLVEKVQAAVGTSAAPVPSDNH

SEQ ID NO: 362 - protein, 261 aa, synthetic construct
FIGITELLKPLGLWASQVTQELRALMDETMKELKAYKSELEEQLTPVAEETRARLSKELQAAQARLGADMEDVCGRLVQYRGEVQAMLGQSTEELRVSLASHLRKLRKRLLRDADDLQKCLAVYQAGAREGAERGLSAIRERLGPLVEQGRVRAATVGSLAGQPLQERAQAWGERLRARMEEMGSRTRDRLDEVKEQVAEVRAKLEEQAQQIRLQAEAFQARLKSWFEPLVEDMQRQWAGLVEKVQAAVGTSAAPVPSDNH

SEQ ID NO: 363 - protein, 265 aa, synthetic construct
FIGITELLKAGNRVRRSVGSQVTQELRALMDETMKELKAYKSELEEQLTPVAEETRARLSKELQAAQARLGADMEDVCGRLVQYRGEVQAMLGQSTEELRVSLASHLRKLRKRLLRDADDLQKCLAVYQAGAREGAERGLSAIRERLGPLVEQGRVRAATVGSLAGQPLQERAQAWGERLRARMEEMGSRTRDRLDEVKEQVAEVRAKLEEQAQQIRLQAEAFQARLKSWFEPLVEDMQRQWAGLVEKVQAAVGTSAAPVPSDNH

SEQ ID NO: 364 - protein, 303 aa, synthetic construct
FIGITELLKGFLGPEPELRQQTEWQSGQRWELALGRFWDYLRWVQTLSEQVQEELLSSQVTQELRALMDETMKELKAYKSELEEQLTPVAEETRARLSKELQAAQARLGADMEDVCGRLVQYRGEVQAMLGQSTEELRVSLASHLRKLRKRLLRDADDLQKCLAVYQAGAREGAERGLSAIRERLGPLVEQGRVRAATVGSLAGQPLQERAQAWGERLRARMEEMGSRTRDRLDEVKEQVAEVRAKLEEQAQQIRLQAEAFQARLKSWFEPLVEDMQRQWAGLVEKVQAAVGTSAAPVPSDNH

SEQ ID NO: 365 - protein, 305 aa, synthetic construct
FIGITELLKPLGLWAPEPELRQQTEWQSGQRWELALGRFWDYLRWVQTLSEQVQEELLSSQVTQELRALMDETMKELKAYKSELEEQLTPVAEETRARLSKELQAAQARLGADMEDVCGRLVQYRGEVQAMLGQSTEELRVSLASHLRKLRKRLLRDADDLQKCLAVYQAGAREGAERGLSAIRERLGPLVEQGRVRAATVGSLAGQPLQERAQAWGERLRARMEEMGSRTRDRLDEVKEQVAEVRAKLEEQAQQIRLQAEAFQARLKSWFEPLVEDMQRQWAGLVEKVQAAVGTSAAPVPSDNH

SEQ ID NO: 366 - protein, 309 aa, synthetic construct
FIGITELLKAGNRVRRSVGPEPELRQQTEWQSGQRWELALGRFWDYLRWVQTLSEQVQEELLSSQVTQELRALMDETMKELKAYKSELEEQLTPVAEETRARLSKELQAAQARLGADMEDVCGRLVQYRGEVQAMLGQSTEELRVSLASHLRKLRKRLLRDADDLQKCLAVYQAGAREGAERGLSAIRERLGPLVEQGRVRAATVGSLAGQPLQERAQAWGERLRARMEEMGSRTRDRLDEVKEQVAEVRAKLEEQAQQIRLQAEAFQARLKSWFEPLVEDMQRQWAGLVEKVQAAVGTSAAPVPSDNH

SEQ ID NO: 367 - protein, 312 aa, synthetic construct
FIGITELHKGFLGKVEQAVETEPEPELRQQTEWQSGQRWELALGRFWDYLRWVQTLSEQVQEELLSSQVTQELRALMDETMKELKAYKSELEEQLTPVAEETRARLSKELQAAQARLGADMEDVCGRLVQYRGEVQAMLGQSTEELRVSLASHLRKLRKRLLRDADDLQKCLAVYQAGAREGAERGLSAIRERLGPLVEQGRVRAATVGSLAGQPLQERAQAWGERLRARMEEMGSRTRDRLDEVKEQVAEVRAKLEEQAQQIRLQAEAFQARLKSWFEPLVEDMQRQWAGLVEKVQAAVGTSAAPVPSDNH

SEQ ID NO: 368 - protein, 314 aa, synthetic construct
FIGITELHKPLGLWAKVEQAVETEPEPELRQQTEWQSGQRWELALGRFWDYLRWVQTLSEQVQEELLSSQVTQELRALMDETMKELKAYKSELEEQLTPVAEETRARLSKELQAAQARLGADMEDVCGRLVQYRGEVQAMLGQSTEELRVSLASHLRKLRKRLLRDADDLQKCLAVYQAGAREGAERGLSAIRERLGPLVEQGRVRAATVGSLAGQPLQERAQAWGERLRARMEEMGSRTRDRLDEVKEQVAEVRAKLEEQAQQIRLQAEAFQARLKSWFEPLVEDMQRQWAGLVEKVQAAVGTSAAPVPSDNH

SEQ ID NO: 369 - protein, 318 aa, synthetic construct
FIGITELHKAGNRVRRSVGKVEQAVETEPEPELRQQTEWQSGQRWELALGRFWDYLRWVQTLSEQVQEELLSSQVTQELRALMDETMKELKAYKSELEEQLTPVAEETRARLSKELQAAQARLGADMEDVCGRLVQYRGEVQAMLGQSTEELRVSLASHLRKLRKRLLRDADDLQKCLAVYQAGAREGAERGLSAIRERLGPLVEQGRVRAATVGSLAGQPLQERAQAWGERLRARMEEMGSRTRDRLDEVKEQVAEVRAKLEEQAQQIRLQAEAFQARLKSWFEPLVEDMQRQWAGLVEKVQAAVGTSAAPVPSDNH

SEQ ID NO: 370 - protein, 122 aa, synthetic construct
FIGITELHKGFLGRAATVGSLAGQPLQERAQAWGERLRARMEEMGSRTRDRLDEVKEQVAEVRAKLEEQAQQIRLQAEAFQARLKSWFEPLVEDMQRQWAGLVEKVQAAVGTSAAPVPSDNH

SEQ ID NO: 371 - protein, 124 aa, synthetic construct
FIGITELHKPLGLWARAATVGSLAGQPLQERAQAWGERLRARMEEMGSRTRDRLDEVKEQVAEVRAKLEEQAQQIRLQAEAFQARLKSWFEPLVEDMQRQWAGLVEKVQAAVGTSAAPVPSDNH

SEQ ID NO: 372 - protein, 128 aa, synthetic construct
FIGITELHKAGNRVRRSVGRAATVGSLAGQPLQERAQAWGERLRARMEEMGSRTRDRLDEVKEQVAEVRAKLEEQAQQIRLQAEAFQARLKSWFEPLVEDMQRQWAGLVEKVQAAVGTSAAPVPSDNH

SEQ ID NO: 373 - protein, 149 aa, synthetic construct
FIGITELHKGFLGAGAREGAERGLSAIRERLGPLVEQGRVRAATVGSLAGQPLQERAQAWGERLRARMEEMGSRTRDRLDEVKEQVAEVRAKLEEQAQQIRLQAEAFQARLKSWFEPLVEDMQRQWAGLVEKVQAAVGTSAAPVPSDNH

SEQ ID NO: 374 - protein, 151 aa, synthetic construct
FIGITELHKPLGLWAAGAREGAERGLSAIRERLGPLVEQGRVRAATVGSLAGQPLQERAQAWGERLRARMEEMGSRTRDRLDEVKEQVAEVRAKLEEQAQQIRLQAEAFQARLKSWFEPLVEDMQRQWAGLVEKVQAAVGTSAAPVPSDNH

SEQ ID NO: 375 - protein, 155 aa, synthetic construct
FIGITELHKAGNRVRRSVGAGAREGAERGLSAIRERLGPLVEQGRVRAATVGSLAGQPLQERAQAWGERLRARMEEMGSRTRDRLDEVKEQVAEVRAKLEEQAQQIRLQAEAFQARLKSWFEPLVEDMQRQWAGLVEKVQAAVGTSAAPVPSDNH

SEQ ID NO: 376 - protein, 269 aa, synthetic construct
FIGITELHKGFLGSEQVQEELLSSQVTQELRALMDETMKELKAYKSELEEQLTPVAEETRARLSKELQAAQARLGADMEDVCGRLVQYRGEVQAMLGQSTEELRVSLASHLRKLRKRLLRDADDLQKCLAVYQAGAREGAERGLSAIRERLGPLVEQGRVRAATVGSLAGQPLQERAQAWGERLRARMEEMGSRTRDRLDEVKEQVAEVRAKLEEQAQQIRLQAEAFQARLKSWFEPLVEDMQRQWAGLVEKVQAAVGTSAAPVPSDNH

SEQ ID NO: 377 - protein, 271 aa, synthetic construct
FIGITELHKPLGLWASEQVQEELLSSQVTQELRALMDETMKELKAYKSELEEQLTPVAEETRARLSKELQAAQARLGADMEDVCGRLVQYRGEVQAMLGQSTEELRVSLASHLRKLRKRLLRDADDLQKCLAVYQAGAREGAERGLSAIRERLGPLVEQGRVRAATVGSLAGQPLQERAQAWGERLRARMEEMGSRTRDRLDEVKEQVAEVRAKLEEQAQQIRLQAEAFQARLKSWFEPLVEDMQRQWAGLVEKVQAAVGTSAAPVPSDNH

SEQ ID NO: 378 - protein, 275 aa, synthetic construct
FIGITELHKAGNRVRRSVGSEQVQEELLSSQVTQELRALMDETMKELKAYKSELEEQLTPVAEETRARLSKELQAAQARLGADMEDVCGRLVQYRGEVQAMLGQSTEELRVSLASHLRKLRKRLLRDADDLQKCLAVYQAGAREGAERGLSAIRERLGPLVEQGRVRAATVGSLAGQPLQERAQAWGERLRARMEEMGSRTRDRLDEVKEQVAEVRAKLEEQAQQIRLQAEAFQARLKSWFEPLVEDMQRQWAGLVEKVQAAVGTSAAPVPSDNH

SEQ ID NO: 379 - protein, 259 aa, synthetic construct
FIGITELHKGFLGSQVTQELRALMDETMKELKAYKSELEEQLTPVAEETRARLSKELQAAQARLGADMEDVCGRLVQYRGEVQAMLGQSTEELRVSLASHLRKLRKRLLRDADDLQKCLAVYQAGAREGAERGLSAIRERLGPLVEQGRVRAATVGSLAGQPLQERAQAWGERLRARMEEMGSRTRDRLDEVKEQVAEVRAKLEEQAQQIRLQAEAFQARLKSWFEPLVEDMQRQWAGLVEKVQAAVGTSAAPVPSDNH

SEQ ID NO: 380 - protein, 261 aa, synthetic construct
FIGITELHKPLGLWASQVTQELRALMDETMKELKAYKSELEEQLTPVAEETRARLSKELQAAQARLGADMEDVCGRLVQYRGEVQAMLGQSTEELRVSLASHLRKLRKRLLRDADDLQKCLAVYQAGAREGAERGLSAIRERLGPLVEQGRVRAATVGSLAGQPLQERAQAWGERLRARMEEMGSRTRDRLDEVKEQVAEVRAKLEEQAQQIRLQAEAFQARLKSWFEPLVEDMQRQWAGLVEKVQAAVGTSAAPVPSDNH

SEQ ID NO: 381 - protein, 265 aa, synthetic construct
FIGITELHKAGNRVRRSVGSQVTQELRALMDETMKELKAYKSELEEQLTPVAEETRARLSKELQAAQARLGADMEDVCGRLVQYRGEVQAMLGQSTEELRVSLASHLRKLRKRLLRDADDLQKCLAVYQAGAREGAERGLSAIRERLGPLVEQGRVRAATVGSLAGQPLQERAQAWGERLRARMEEMGSRTRDRLDEVKEQVAEVRAKLEEQAQQIRLQAEAFQARLKSWFEPLVEDMQRQWAGLVEKVQAAVGTSAAPVPSDNH

SEQ ID NO: 382 - protein, 303 aa, synthetic construct
FIGITELHKGFLGPEPELRQQTEWQSGQRWELALGRFWDYLRWVQTLSEQVQEELLSSQVTQELRALMDETMKELKAYKSELEEQLTPVAEETRARLSKELQAAQARLGADMEDVCGRLVQYRGEVQAMLGQSTEELRVSLASHLRKLRKRLLRDADDLQKCLAVYQAGAREGAERGLSAIRERLGPLVEQGRVRAATVGSLAGQPLQERAQAWGERLRARMEEMGSRTRDRLDEVKEQVAEVRAKLEEQAQQIRLQAEAFQARLKSWFEPLVEDMQRQWAGLVEKVQAAVGTSAAPVPSDNH

SEQ ID NO: 383 - protein, 305 aa, synthetic construct
FIGITELHKPLGLWAPEPELRQQTEWQSGQRWELALGRFWDYLRWVQTLSEQVQEELLSSQVTQELRALMDETMKELKAYKSELEEQLTPVAEETRARLSKELQAAQARLGADMEDVCGRLVQYRGEVQAMLGQSTEELRVSLASHLRKLRKRLLRDADDLQKCLAVYQAGAREGAERGLSAIRERLGPLVEQGRVRAATVGSLAGQPLQERAQAWGERLRARMEEMGSRTRDRLDEVKEQVAEVRAKLEEQAQQIRLQAEAFQARLKSWFEPLVEDMQRQWAGLVEKVQAAVGTSAAPVPSDNH

SEQ ID NO: 384 - protein, 309 aa, synthetic construct
FIGITELHKAGNRVRRSVGPEPELRQQTEWQSGQRWELALGRFWDYLRWVQTLSEQVQEELLSSQVTQELRALMDETMKELKAYKSELEEQLTPVAEETRARLSKELQAAQARLGADMEDVCGRLVQYRGEVQAMLGQSTEELRVSLASHLRKLRKRLLRDADDLQKCLAVYQAGAREGAERGLSAIRERLGPLVEQGRVRAATVGSLAGQPLQERAQAWGERLRARMEEMGSRTRDRLDEVKEQVAEVRAKLEEQAQQIRLQAEAFQARLKSWFEPLVEDMQRQWAGLVEKVQAAVGTSAAPVPSDNH

SEQ ID NO: 385 - protein, 12 aa, synthetic construct
KVEQAVETEPEP

SEQ ID NO: 386 - protein, 14 aa, synthetic construct
TLSEQVQEELLSSQ

SEQ ID NO: 387 - protein, 27 aa, synthetic construct
ELRVRLASHLRKLRKRLLRDADDLQKC

SEQ ID NO: 388 - protein, 40 aa, synthetic construct
YQAGAREGAERGLSAIRERLGPLVEQGRVRAATVGSLAGQ

SEQ ID NO: 389 - protein, 299 aa, synthetic construct
KVEQAVETEPEPELRQQTEWQSGQRWELALGRFWDYLRWVQTLSEQVQEELLSSQVTQELTALMDETMKELKAYKSELEEQLTPVAEETRARLSKELQAAQARLGADMEDVCGRLVQYRGEVQAMLGQSTEELRVRLASHLRKLRKRLLRDADDLQKCLAVYQAGAREGAERGLSAIRERLGPLVEQGRVRAATVGSLAGQPLQERAQAWGERLRARMEEMGSRTRDRLDEVKEQVAEVRAKLEEQAQQIRLQAEAFQARLKSWFEPLVEDMQRQWAGLVEKVQAAVGTSAAPVPSDNH

SEQ ID NO: 390 - protein, 299 aa, synthetic construct; identical to SEQ ID NO: 18

SEQ ID NO: 391 - protein, 299 aa, synthetic construct
KVEQAVETEPEPELRQQTEWQSGQRWELALGRFWDYLRWVQTLSEQVQEELLSSQVTQELRALMDETMKELKAYKSELEEQLTPVAEETRARLSKELQAAQARLGADMEDVCGRLVQYRGEVQAMLGQSTEELRVRLASALRKLRKRLLRDADDLQKCLAVYQAGAREGAERGLSAIRERLGPLVEQGRVRAATVGSLAGQPLQERAQAWGERLRARMEEMGSRTRDRLDEVKEQVAEVRAKLEEQAQQIRLQAEAFQARLKSWFEPLVEDMQRQWAGLVEKVQAAVGTSAAPVPSDNH

SEQ ID NO: 392 - protein, 299 aa, synthetic construct
KVEQAVETEPEPELRQQTEWQSGQRWELALGRFWDYLRWVQTLSEQVQEELLSSQVTQELRALMDETMKELKAYKSELEEQLTPVAEETRARLSKELQAAQARLGADMEDVCGRLVQYRGEVQAMLGQSTEELRVRLASHLRALRKRLLRDADDLQKCLAVYQAGAREGAERGLSAIRERLGPLVEQGRVRAATVGSLAGQPLQERAQAWGERLRARMEEMGSRTRDRLDEVKEQVAEVRAKLEEQAQQIRLQAEAFQARLKSWFEPLVEDMQRQWAGLVEKVQAAVGTSAAPVPSDNH

SEQ ID NO: 393 - protein, 299 aa, synthetic construct
KVEQAVETEPEPELRQQTEWQSGQRWELALGRFWDYLRWVQTLSEQVQEELLSSQVTQELRALMDETMKELKAYKSELEEQLTPVAEETRARLSKELQAAQARLGADMEDVCGRLVQYRGEVQAMLGQSTEELRVRLASHLRKPRKRLLRDADDLQKCLAVYQAGAREGAERGLSAIRERLGPLVEQGRVRAATVGSLAGQPLQERAQAWGERLRARMEEMGSRTRDRLDEVKEQVAEVRAKLEEQAQQIRLQAEAFQARLKSWFEPLVEDMQRQWAGLVEKVQAAVGTSAAPVPSDNH

SEQ ID NO: 394 - protein, 299 aa, synthetic construct
KVEQAVETEPEPELRQQTEWQSGQRWELALGRFWDYLRWVQTLSEQVQEELLSSQVTQELRALMDETMKELKAYKSELEEQLTPVAEETRARLSKELQAAQARLGADMEDVCGRLVQYRGEVQAMLGQSTEELRVRLASHLRKLRKRLLADADDLQKCLAVYQAGAREGAERGLSAIRERLGPLVEQGRVRAATVGSLAGQPLQERAQAWGERLRARMEEMGSRTRDRLDEVKEQVAEVRAKLEEQAQQIRLQAEAFQARLKSWFEPLVEDMQRQWAGLVEKVQAAVGTSAAPVPSDNH

SEQ ID NO: 395 - protein, 299 aa, synthetic construct
KVEQAVETEPEPELRQQTEWQSGQRWELALGRFWDYLRWVQTLSEQVQEELLSSQVTQELRALMDETMKELKAYKSELEEQLTPVAEETRARLSKELQAAQARLGADMEDVCGRLVQYRGEVQAMLGQSTEELRVSLASALRKLRKRLLRDADDLQKCLAVYQAGAREGAERGLSAIRERLGPLVEQGRVRAATVGSLAGQPLQERAQAWGERLRARMEEMGSRTRDRLDEVKEQVAEVRAKLEEQAQQIRLQAEAFQARLKSWFEPLVEDMQRQWAGLVEKVQAAVGTSAAPVPSDNH

SEQ ID NO: 396 - protein, 299 aa, synthetic construct
KVEQAVETEPEPELRQQTEWQSGQRWELALGRFWDYLRWVQTLSEQVQEELLSSQVTQELRALMDETMKELKAYKSELEEQLTPVAEETRARLSKELQAAQARLGADMEDVCGRLVQYRGEVQAMLGQSTEELRVSLASHLRKPRKRLLRDADDLQKCLAVYQAGAREGAERGLSAIRERLGPLVEQGRVRAATVGSLAGQPLQERAQAWGERLRARMEEMGSRTRDRLDEVKEQVAEVRAKLEEQAQQIRLQAEAFQARLKSWFEPLVEDMQRQWAGLVEKVQAAVGTSAAPVPSDNH

SEQ ID NO: 397 - protein, 299 aa, synthetic construct
KVEQAVETEPEPELRQQTEWQSGQRWELALGRFWDYLRWVQTLSEQVQEELLSSQVTQELRALMDETMKELKAYKSELEEQLTPVAEETRARLSKELQAAQARLGADMEDVCGRLVQYRGEVQAMLGQSTEELRVSLASALRKPRKRLLRDADDLQKCLAVYQAGAREGAERGLSAIRERLGPLVEQGRVRAATVGSLAGQPLQERAQAWGERLRARMEEMGSRTRDRLDEVKEQVAEVRAKLEEQAQQIRLQAEAFQARLKSWFEPLVEDMQRQWAGLVEKVQAAVGTSAAPVPSDNH

SEQ ID NO: 398 - protein, 299 aa, synthetic construct
KVEQAVETEPEPELRQQTEWQSGQRWELALGRFWDYLRWVQTLSEQVQEELLSSQVTQELRALMDETMKELKAYKSELEEQLTPVAEETRARLSKELQAAQARLGADMEDVCGRLVQYRGEVQAMLGQSTEELRVSLASHLRALRKRLLRDADDLQKCLAVYQAGAREGAERGLSAIRERLGPLVEQGRVRAATVGSLAGQPLQERAQAWGERLRARMEEMGSRTRDRLDEVKEQVAEVRAKLEEQAQQIRLQAEAFQARLKSWFEPLVEDMQRQWAGLVEKVQAAVGTSAAPVPSDNH

SEQ ID NO: 399 - protein, 299 aa, synthetic construct
KVEQAVETEPEPELRQQTEWQSGQRWELALGRFWDYLRWVQTLSEQVQEELLSSQVTQELRALMDETMKELKAYKSELEEQLTPVAEETRARLSKELQAAQARLGADMEDVCGRLVQYRGEVQAMLGQSTEELRVSLASHLRKLRKRLLADADDLQKCLAVYQAGAREGAERGLSAIRERLGPLVEQGRVRAATVGSLAGQPLQERAQAWGERLRARMEEMGSRTRDRLDEVKEQVAEVRAKLEEQAQQIRLQAEAFQARLKSWFEPLVEDMQRQWAGLVEKVQAAVGTSAAPVPSDNH

SEQ ID NO: 400 - protein, 299 aa, synthetic construct
KVEQAVETEPEPELRQQTEWQSGQRWELALGRFWDYLRWVQTLSEQVQEELLSSQVTQELRALMDETMKELKAYKSELEEQLTPVAEETRARLSKELQAAQARLGADMEDVCGRLVQYRGEVQAMLGQSTEELRVSLASHLRALRKRLLADADDLQKCLAVYQAGAREGAERGLSAIRERLGPLVEQGRVRAATVGSLAGQPLQERAQAWGERLRARMEEMGSRTRDRLDEVKEQVAEVRAKLEEQAQQIRLQAEAFQARLKSWFEPLVEDMQRQWAGLVEKVQAAVGTSAAPVPSDNH

SEQ ID NO: 401 - protein, 299 aa, synthetic construct
KVEQAVETEPEPELRQQTEWQSGQRWELALGRFWDYLRWVQTLSEQVQEELLSSQVTQELTALMDETMKELKAYKSELEEQLTPVAEETRARLSKELQAAQARLGADMEDVCGRLVQYRGEVQAMLGQSTEELRVSLASHLRKLRKRLLRDADDLQKCLAVYQAGAREGAERGLSAIRERLGPLVEQGRVRAATVGSLAGQPLQERAQAWGERLRARMEEMGSRTRDRLDEVKEQVAEVRAKLEEQAQQIRLQAEAFQARLKSWFEPLVEDMQRQWAGLVEKVQAAVGTSAAPVPSDNH

SEQ ID NO: 402 - protein, 249 aa, synthetic construct
RHFWQQDEPPQSPWDRVKDLATVYVDVLKDSGRDYVSQFEGSALGKQLNLKLLDNWDSVTSTFSKLREQLGPVTQEFWDNLEKETEGLRQEMSKDLEEVKAKVQPYLDDFQKKWQEEMELYRQKVEPLRAELQEGARQKLHELQEKLSPLGEEMRDRARAHVDALRTHLAPYSDELRQRLAARLEALKENGGARLAEYHAKATEHLSTLSEKAKPALEDLRQGLLPVLESFKVSFLSALEEYTKKLNTQ

SEQ ID NO: 403 - protein, 82 aa, synthetic construct
ALVRRQAKEPCVESLVSQYFQTVTDYGKDLMEKVKSPELQAEAKSYFEKSKEQLTPLIKKAGTELVNFLSYFVELGTQPATQ

SEQ ID NO: 404 - protein, 376 aa, synthetic construct
EVSADQVATVMWDYFSQLSNNAKEAVEHLQKSELTQQLNALFQDKLGEVNTYAGDLQKKLVPFATELHERLAKDSEKLKEEIGKELEELRARLLPHANEVSQKIGDNLRELQQRLEPYADQLRTQVSTQAEQLRRQLTPYAQRMERVLRENADSLQASLRPHADELKAKIDQNVEELKGRLTPYADEFKVKIDQTVEELRRSLAPYAQDTQEKLNHQLEGLTFQMKKNAEELKARISASAEELRQRLAPLAEDVRGNLRGNTEGLQKSLAELGGHLDQQVEEFRRRVEPYGENFNKALVQQMEQLRQKLGPHAGDVEGHLSFLEKDLRDKVNSFFSTFKEKESQDKTLSLPELEQQQEQQQEQQQEQVQMLAPLES

SEQ ID NO: 405 - protein, 343 aa, synthetic construct
RKGFWDYFSQTSGDKGRVEQIHQQKMAREPATLKDSLEQDLNNMNKFLEKLRPLSGSEAPRLPQDPVGMRRQLQEELEEVKARLQPYMAEAHELVGWNLEGLRQQLKPYTMDLMEQVALRVQELQEQLRVVGEDTKAQLLGGVDEAWALLQGLQSRVVHHTGRFKELFHPYAESLVSGIGRHVQELHRSVAPHAPASPARLSRCVQVLSRKLTLKAKALHARIQQNLDQLREELSRAFAGTGTEEGAGPDPQMLSEEVRQRLQAFRQDTYLQIAAFTRAIDQETEEVQQQLAPPPPGHSAFAPEFQQTDSGKVLSKLQARLDDLWEDITHSLHDQGHSHLGDP

SEQ ID NO: 406 - protein, 1097 aa, synthetic construct
MDFLRLYLPGLHQALRGALDSLGTFVSYLLGDAVPTVEREAQAAEELGVVAVGKTGKIVEEEAQEDLEGLRGSQNEGAGRLRGPGDDRRHEVGSSAVEQTWGWGDGSSHGSQAERQDSGAGETAKAARCQEPSAHLEARKKSKAGSGACQDRSGQAQERQESHEQEVNREERLRSWEQEEEEEEVRAREPGMARGAESEWTWHGETEGKAGAVGPKAAGDNREMEQGVREADAGETEEPGAEGAGKGEEVVVVEKACESTRAWGTWGPGAEPEDWGILGREEARTTPGREEARAILDGEEARTISGGEEAETASGGEEAETASGGEEAGTASGGEEAGIASGGEAGTASGGEEAGTASGGEEAGTASGGDEAWTTSGKEEADLLGVRQTEYGAVPGERLLEATGKVWVLEEEGDEEREAEVSPFPKQPQVLGTERTEEAAESQTAGREAVGGQEAGESFEGQVDLRGKEAEMRQDLGIRADRARMEELVQAEEAQEERGSSRDPVAELPSDGEAEGTADLEATPEARPEEELTGEESEAAQTSCGLLGVEWGGLTHSVTKGQGPELMGGAQTPTKQPEEREAGEVELMGVLALSKEEQERSLEAGPRHAGSVKPEASEAFPGAWENRTRKDMERGNTQEDAADGEQREEEETAGGQTLAAEAEGDRESELSEVPEAGGEGLTTQDAGCGTEEGEASVSENQELDGSTGADAGPCPSLGEAYARETEDEEAEADRTSRRGWRLQAVAVGLPDREDAQTGSVAAGIMGGDVVPHISAAGAGEALEGVLGQGWDSKEKEEAAAGEHAGGQEFGLEGSAEEEVTGRGSQVEAFESREGGPWGGRVEAEESAGAEDSCGLDPAGSQTARAEGMGAMVEAGGLLEKWTLLEEEAVGWQEREQREDSEGRCGDYHPEGEAPRLLDAEGLMVTGGRRAEAKETEPESLEHVRGQEEQPTHQAPAEAAPESVGEAETAEAMGSARGGAANSWSEAPLPGSLLDVSVPRSRVHLSRSSSQRRSRPSFRRTPAWEQQEEPPAPNPPEEELSAPEQRPLQLEEPLEPSPLRHDGTPVPARRRPLGHGFGLAHPGMMQELQARLGRPKPQ

SEQ ID NO: 407 - protein, 57 aa, synthetic construct
TPDVSSALDKLKEFGNTLEDKARELISRIKQSELSAKMREWFSETFQKVKEKLKIDS

SEQ ID NO: 408 - protein, 79 aa, synthetic construct
TQQPQQDEMPSPTFLTQVKESLSSYWESAKTAAQNLYEKTYLPAVDEKLRDLYSKSTAAMSTYTGIFTDQVLSVLKGEE

SEQ ID NO: 409 - protein, 79 aa, synthetic construct
SEAEDASLLSFMQGYMKHATKTAKDALSSVQESQVAQQARGWVTDGFSSLKDYWSTVKDKFSEFWDLDPEVRPTSAVAA

SEQ ID NO: 410 - protein, 100 aa, synthetic construct
QPEAQEGTLSPPPKLKMSRWSLVRGRMKELLETVVNRTRDGWQWFWSPSTFRGFMQTYYDDHLRDLGPLTKAWFLESKDSLLKKTHSLCPRLVCGDKDQG

SEQ ID NO: 411 - protein, 169 aa, synthetic construct
QAFHLGKCPNPPVQENFDVNKYLGRWYEIEKIPTTFENGRCIQANYSLMENGKIKVLNQELRADGTVNQIEGEATPVNLTEPAKLEVKFSWFMPSAPYWILATDYENYALVYSCTCIIQLFHVDFAWILARNPNLPPETVDSLKNILTSNNIDVKKMTVTDQVNCPKLS

SEQ ID NO: 412 - protein, 326 aa, synthetic construct
GRTCPKPDDLPFSTVVPLKTFYEPGEEITYSCKPGYVSRGGMRKFICPLTGLWPINTLKCTPRVCPFAGILENGAVRYTTFEYPNTISFSCNTGFYLNGADSAKCTEEGKWSPELPVCAPIICPPPSIPTFATLRVYKPSAGNNSLYRDTAVFECLPQHAMFGNDTITCTTHGNWTKLPECREVKCPFPSRPDNGFVNYPAKPTLYYKDKATFGCHDGYSLDGPEEIECTKLGNWSAMPSCKASCKVPVKKATVVYQGERVKIQEKFKNGMLHGDKVSFFCKNKEKKCSYTEDAQCIDGTIEVPKCFKEHSSLAFWKTDASDVKPC

SEQ ID NO: 413 - protein, 166 aa, synthetic construct
CPEHSQLTTLGVDGKEFPEVHLGQWYFIAGAAPTKEELATFDPVDNIVFNMAAGSAPMQLHLRATIRMKDGLCVPRKWIYHLTEGSTDLRTEGRPDMKTELFSSSCPGGIMLNETGQGYQRFLLYNRSPHPPEKCVEEFKSLTSCLDSKAFLLTPRNQEACELSNN

SEQ ID NO: 414 - protein, 5 aa, synthetic construct
SSSSG

SEQ ID NO: 415 - protein, 16 aa, synthetic construct
GGGGSLVPRGSGGGGS

SEQ ID NO: 416 - protein, 6 aa, synthetic construct
GSGSGS

SEQ ID NO: 417 - protein, 8 aa, synthetic construct
GSGSGSGS

SEQ ID NO: 418 - protein, 12 aa, synthetic construct
GSGSGSGSGSGS

SEQ ID NO: 419 - protein, 11 aa, synthetic construct
GGSGGHMGSGG

SEQ ID NO: 420 - protein, 11 aa, synthetic construct
GGSGGSGGSGG

SEQ ID NO: 421 - protein, 5 aa, synthetic construct
GGSGG

SEQ ID NO: 422 - protein, 8 aa, synthetic construct
GGSGGGGG

SEQ ID NO: 423 - protein, 18 aa, synthetic construct
GGGSEGGGSEGGGSEGGG

SEQ ID NO: 424 - protein, 8 aa, synthetic construct
AAGAATAA

SEQ ID NO: 425 - protein, 5 aa, synthetic construct
GGGGG

SEQ ID NO: 426 - protein, 5 aa, synthetic construct
GGSSG

SEQ ID NO: 427 - protein, 11 aa, synthetic construct
GSGGGTGGGSG

SEQ ID NO: 428 - protein, 11 aa, synthetic construct
GSGGGTGGGSG

SEQ ID NO: 429 - protein, 12 aa, synthetic construct
GSGSGSGSGGSG

SEQ ID NO: 430 - protein, 14 aa, synthetic construct
GSGGSGGSGGSGGS

SEQ ID NO: 431 - protein, 14 aa, synthetic construct
GSGGSGSGGSGGSG

SEQ ID NO: 432 - protein, 15 aa, synthetic construct
SSSSGSSSSGSSSSG

SEQ ID NO: 433 - protein, 20 aa, synthetic construct
SSSSGSSSSGSSSSGSSSSG

SEQ ID NO: 434 - protein, 4 aa, synthetic construct
GTGT

SEQ ID NO: 435 - protein, 6 aa, synthetic construct
GTGTGT

SEQ ID NO: 436 - protein, 245 aa, synthetic construct
QVQLVQSGAEVKKPGASVKVSCKASGFNIKDFNIHWVRQAPGQGLEWIGRIDPESGDAEYVPKFQGRVTMTRDTSTSTVYMELSSLRSEDTAVYYCTTGSYDLDVEYWGQGTLVTVSSGGGGSGGGGSGGGGSGGGGSDIQMTQSPSSLSASVGDRVTITCHASQNINVWLSWYQQKPGKAPKLLIYKASTLHTGVPSRFSGSGSGTDFTLTISSLQPEDFATYYCQQGQSYPLTFGQGTKLEIK

SEQ ID NO: 437 - protein, 245 aa, synthetic construct
QVQLVQSGAEVKKPGASVKVSCKASGFNIKDFNIHWVRQAPGQGLEWIGRIDPEGGDAEYVPKFQGRVTMTRDTSTSTVYMELSSLRSEDTAVYYCTTGSYDLDVEYWGQGTLVTVSSGGGGSGGGGSGGGGSGGGGSDIQMTQSPSSLSASVGDRVTITCHASQNINVWLSWYQQKPGKAPKLLIYKASTLHTGVPSRFSGSGSGTDFTLTISSLQPEDFATYYCQQGQSYPLTFGQGTKLEIK

SEQ ID NO: 438 - protein, 245 aa, synthetic construct
QVQLVQSGAEVKKPGASVKVSCKASGFNIKDFNIHWVRQAPGQGLEWIGRIDPEQGDAEYVPKFQGRVTMTRDTSTSTVYMELSSLRSEDTAVYYCTTGSYDLDVEYWGQGTLVTVSSGGGGSGGGGSGGGGSGGGGSDIQMTQSPSSLSASVGDRVTITCHASQNINVWLSWYQQKPGKAPKLLIYKASTLHTGVPSRFSGSGSGTDFTLTISSLQPEDFATYYCQQGQSYPLTFGQGTKLEIK

SEQ ID NO: 439 - protein, 245 aa, synthetic construct
QVQLVQSGAEVKKPGASVKVSCKASGFNIKDFNIHWVRQAPGQGLEWIGRIDPEDGDAEYVPKFQGRVTMTRDTSTSTVYMELSSLRSEDTAVYYCTTGSYDLDVEYWGQGTLVTVSSGGGGSGGGGSGGGGSGGGGSDIQMTQSPSSLSASVGDRVTITCHASQNINVWLSWYQQKPGKAPKLLIYKASTLHTGVPSRFSGSGSGTDFTLTISSLQPEDFATYYCQQGQSYPLTFGQGTKLEIK

SEQ ID NO: 440 - protein, 245 aa, synthetic construct
QVQLVQSGAEVKKPGASVKVSCKASGFNIKDFNIHWVRQAPGQGLEWIGRIDPENADAEYVPKFQGRVTMTRDTSTSTVYMELSSLRSEDTAVYYCTTGSYDLDVEYWGQGTLVTVSSGGGGSGGGGSGGGGSGGGGSDIQMTQSPSSLSASVGDRVTITCHASQNINVWLSWYQQKPGKAPKLLIYKASTLHTGVPSRFSGSGSGTDFTLTISSLQPEDFATYYCQQGQSYPLTFGQGTKLEIK

SEQ ID NO: 441 - protein, 245 aa, synthetic construct
QVQLVQSGAEVKKPGASVKVSCKASGFNIKDFNIHWVRQAPGQGLEWIGRIDPENGDAEYVPKFQGRVTMTRDTSTSTVYMELSSLRSEDTAVYYCTTGSYDLDVEYWGQGTLVTVSSGGGGSGGGGSGGGGSGGGGSDIQMTQSPSSLSASVGDRVTITCHASQNINVWLSWYQQKPGKAPKLLIYKASTLHTGVPSRFSGSGSGTDFTLTISSLQPEDFATYYCQQGQSYPLTFGQGTKLEIK

SEQ ID NO: 442 - protein, 214 aa, synthetic construct
DIQMTQSPSSLSASVGDRVTITCRASQSISSYLNWYQQKPGKAPKLLIYAASFLQSGVPSRFSGSGSGTDFTLTISSLQPEDFATYYCQQGYPYPFTFGQGTKLEIKRTVAAPSVFIFPPSDEQLKSGTASVVCLLNNFYPREAKVQWKVDNALQSGNSQESVTEQDSKDSTYSLSSTLTLSKADYEKHKVYACEVTHQGLSSPVTKSFNRGEC

SEQ ID NO: 443 - protein, 447 aa, synthetic construct
EVQLLESGGGLVQPGGSLRLSCAASGFTFSSYAMSWVRQAPGKGLEWVSGISGYSGSTYYADSVKGRFTISRDNSKNTLYLQMNSLRAEDTAVYYCARYYSYYGYYYFDYWGQGTLVTVSSASTKGPSVFPLAPCSRSTSESTAALGCLVKDYFPEPVTVSWNSGALTSGVHTFPAVLQSSGLYSLSSVVTVPSSNFGTQTYTCNVDHKPSNTKVDKTVERKCCVECPPCPAPPVAGPSVFLFPPKPKDTLMISRTPEVTCVVVDVSHEDPEVQFNWYVDGVEVHNAKTKPREEQFNSTFRVVSVLTVVHQDWLNGKEYKCKVSNKGLPAPIEKTISKTKGQPREPQVYTLPPSREEMTKNQVSLTCLVKGFYPSDIAVEWESNGQPENNYKTTPPMLDSDGSFFLYSKLTVDKSRWQQGNVFSCSVMHEALHNHYTQKSLSLSPGK

SEQ ID NO: 444 - protein, 20 aa, synthetic construct
GGGGSGGGGSGGGGSGGGGS

SEQ ID NO: 445 - protein, 25 aa, synthetic construct
GGGGSGGGGSGGGGSGGGGSGGGGS

SEQ ID NO: 446 - protein, 702 aa, synthetic construct
EVQLLESGGGLVQPGGSLRLSCAASGFTFSSYAMSWVRQAPGKGLEWVSGISGYSGSTYYADSVKGRFTISRDNSKNTLYLQMNSLRAEDTAVYYCARYYSYYGYYYFDYWGQGTLVTVSSASTKGPSVFPLAPCSRSTSESTAALGCLVKDYFPEPVTVSWNSGALTSGVHTFPAVLQSSGLYSLSSVVTVPSSNFGTQTYTCNVDHKPSNTKVDKTVERKCCVECPPCPAPPVAGPSVFLFPPKPKDTLMISRTPEVTCVVVDVSHEDPEVQFNWYVDGVEVHNAKTKPREEQFNSTFRVVSVLTVVHQDWLNGKEYKCKVSNKGLPAPIEKTISKTKGQPREPQVYTLPPSREEMTKNQVSLTCLVKGFYPSDIAVEWESNGQPENNYKTTPPMLDSDGSFFLYSKLTVDKSRWQQGNVFSCSVMHEALHNHYTQKSLSLSPGKGGGGSGGGGSQVQLVQSGAEVKKPGASVKVSCKASGFNIKDFNIHWVRQAPGQGLEWIGRIDPESGDAEYVPKFQGRVTMTRDTSTSTVYMELSSLRSEDTAVYYCTTGSYDLDVEYWGQGTLVTVSSGGGGSGGGGSGGGGSGGGGSDIQMTQSPSSLSASVGDRVTITCHASQNINVWLSWYQQKPGKAPKLLIYKASTLHTGVPSRFSGSGSGTDFTLTISSLQPEDFATYYCQQGQSYPLTFGQGTKLEIK

SEQ ID NO: 447 - protein, 11 aa, synthetic construct
  SITE 11: note = AlexaFluor 488 (AF488) conjugated to C-terminal Cys at position 11
FIGITELKKGC

SEQ ID NO: 448 - protein, 450 aa, synthetic construct
EVQLVESGGGLVQPGGSLRLSCAASGFNIKDTYIHWVRQAPGKGLEWVARIYPTNGYTRYADSVKGRFTISADTSKNTAYLQMNSLRAEDTAVYYCSRWGGDGFYAMDYWGQGTLVTVSSASTKGPSVFPLAPSSKSTSGGTAALGCLVKDYFPEPVTVSWNSGALTSGVHTFPAVLQSSGLYSLSSVVTVPSSSLGTQTYICNVNHKPSNTKVDKKVEPKSCDKTHTCPPCPAPELLGGPSVFLFPPKPKDTLMISRTPEVTCVVVDVSHEDPEVKFNWYVDGVEVHNAKTKPREEQYNSTYRVVSVLTVLHQDWLNGKEYKCKVSNKALPAPIEKTISKAKGQPREPQVYTLPPSRDELTKNQVSLTCLVKGFYPSDIAVEWESNGQPENNYKTTPPVLDSDGSFFLYSKLTVDKSRWQQGNVFSCSVMHEALHNHYTQKSLSLSPGK

SEQ ID NO: 449 - protein, 214 aa, synthetic construct
DIQMTQSPSSLSASVGDRVTITCRASQDVNTAVAWYQQKPGKAPKLLIYSASFLYSGVPSRFSGSRSGTDFTLTISSLQPEDFATYYCQQHYTTPPTFGQGTKVEIKRTVAAPSVFIFPPSDEQLKSGTASVVCLLNNFYPREAKVQWKVDNALQSGNSQESVTEQDSKDSTYSLSSTLTLSKADYEKHKVYACEVTHQGLSSPVTKSFNRGEC

SEQ ID NO: 450 - protein, 705 aa, synthetic construct
EVQLVESGGGLVQPGGSLRLSCAASGFNIKDTYIHWVRQAPGKGLEWVARIYPTNGYTRYADSVKGRFTISADTSKNTAYLQMNSLRAEDTAVYYCSRWGGDGFYAMDYWGQGTLVTVSSASTKGPSVFPLAPSSKSTSGGTAALGCLVKDYFPEPVTVSWNSGALTSGVHTFPAVLQSSGLYSLSSVVTVPSSSLGTQTYICNVNHKPSNTKVDKKVEPKSCDKTHTCPPCPAPELLGGPSVFLFPPKPKDTLMISRTPEVTCVVVDVSHEDPEVKFNWYVDGVEVHNAKTKPREEQYNSTYRVVSVLTVLHQDWLNGKEYKCKVSNKALPAPIEKTISKAKGQPREPQVYTLPPSRDELTKNQVSLTCLVKGFYPSDIAVEWESNGQPENNYKTTPPVLDSDGSFFLYSKLTVDKSRWQQGNVFSCSVMHEALHNHYTQKSLSLSPGKGGGGSGGGGSQVQLVQSGAEVKKPGASVKVSCKASGFNIKDFNIHWVRQAPGQGLEWIGRIDPESGDAEYVPKFQGRVTMTRDTSTSTVYMELSSLRSEDTAVYYCTTGSYDLDVEYWGQGTLVTVSSGGGGSGGGGSGGGGSGGGGSDIQMTQSPSSLSASVGDRVTITCHASQNINVWLSWYQQKPGKAPKLLIYKASTLHTGVPSRFSGSGSGTDFTLTISSLQPEDFATYYCQQGQSYPLTFGQGTKLEIK

SEQ ID NO: 451 - protein, 451 aa, synthetic construct
QVQLQQPGAELVKPGASVKMSCKASGYTFTSYNMHWVKQTPGRGLEWIGAIYPGNGDTSYNQKFKGKATLTADKSSSTAYMQLSSLTSEDSAVYYCARSTYYGGDWYFNVWGAGTTVTVSAASTKGPSVFPLAPSSKSTSGGTAALGCLVKDYFPEPVTVSWNSGALTSGVHTFPAVLQSSGLYSLSSVVTVPSSSLGTQTYICNVNHKPSNTKVDKKVEPKSCDKTHTCPPCPAPELLGGPSVFLFPPKPKDTLMISRTPEVTCVVVDVSHEDPEVKFNWYVDGVEVHNAKTKPREEQYNSTYRVVSVLTVLHQDWLNGKEYKCKVSNKALPAPIEKTISKAKGQPREPQVYTLPPSRDELTKNQVSLTCLVKGFYPSDIAVEWESNGQPENNYKTTPPVLDSDGSFFLYSKLTVDKSRWQQGNVFSCSVMHEALHNHYTQKSLSLSPGK

SEQ ID NO: 452 - protein, 213 aa, synthetic construct
QIVLSQSPAILSASPGEKVTMTCRASSSVSYIHWFQQKPGSSPKPWIYATSNLASGVPVRFSGSGSGTSYSLTISRVEAEDAATYYCQQWTSNPPTFGGGTKLEIKRTVAAPSVFIFPPSDEQLKSGTASVVCLLNNFYPREAKVQWKVDNALQSGNSQESVTEQDSKDSTYSLSSTLTLSKADYEKHKVYACEVTHQGLSSPVTKSFNRGEC

SEQ ID NO: 453 - protein, 706 aa, synthetic construct
QVQLQQPGAELVKPGASVKMSCKASGYTFTSYNMHWVKQTPGRGLEWIGAIYPGNGDTSYNQKFKGKATLTADKSSSTAYMQLSSLTSEDSAVYYCARSTYYGGDWYFNVWGAGTTVTVSAASTKGPSVFPLAPSSKSTSGGTAALGCLVKDYFPEPVTVSWNSGALTSGVHTFPAVLQSSGLYSLSSVVTVPSSSLGTQTYICNVNHKPSNTKVDKKVEPKSCDKTHTCPPCPAPELLGGPSVFLFPPKPKDTLMISRTPEVTCVVVDVSHEDPEVKFNWYVDGVEVHNAKTKPREEQYNSTYRVVSVLTVLHQDWLNGKEYKCKVSNKALPAPIEKTISKAKGQPREPQVYTLPPSRDELTKNQVSLTCLVKGFYPSDIAVEWESNGQPENNYKTTPPVLDSDGSFFLYSKLTVDKSRWQQGNVFSCSVMHEALHNHYTQKSLSLSPGKGGGGSGGGGSQVQLVQSGAEVKKPGASVKVSCKASGFNIKDFNIHWVRQAPGQGLEWIGRIDPESGDAEYVPKFQGRVTMTRDTSTSTVYMELSSLRSEDTAVYYCTTGSYDLDVEYWGQGTLVTVSSGGGGSGGGGSGGGGSGGGGSDIQMTQSPSSLSASVGDRVTITCHASQNINVWLSWYQQKPGKAPKLLIYKASTLHTGVPSRFSGSGSGTDFTLTISSLQPEDFATYYCQQGQSYPLTFGQGTKLEIK